European Patent Application EP 4 155 318 A1, published March 29, 2023. Title: BISPECIFIC ANTIBODY AND USE THEREOF. Applicant: HARBOUR BIOMED US, INC. Application EP21832260.0. The sequence listing filed with the application follows.

SEQUENCE LISTING (291 sequences)

SEQ ID NO: 1 - protein, 25 aa, Artificial Sequence
  PR000157 HFWR1 Chothia
EVQLVQSGAEVKKPGASVKVSCKAS

SEQ ID NO: 2 - protein, 25 aa, Artificial Sequence [sequence omitted]

SEQ ID NO: 3 - protein, 25 aa, Artificial Sequence
  PR000483 HFWR1 Chothia
EVQLVQSGAEVKKPGESLRISCKGS

SEQ ID NO: 4 - protein, 25 aa, Artificial Sequence
  PR001476 HFWR1 Chothia, PR002408 HFWR1 Chothia
QVQLVESGGGVVQPGRSLRLSCAAS

SEQ ID NO: 5 - protein, 25 aa, Artificial Sequence
  PR001758 HFWR1 Chothia, PR001781 HFWR1 Chothia
EVQLLESGGGLVQLGGSLRLSCAAS

SEQ ID NO: 6 - protein, 25 aa, Artificial Sequence
  PR001760 HFWR1 Chothia
EVQLVESGGGVVQPGGSLRLSCAAS

SEQ ID NO: 7 - protein, 25 aa, Artificial Sequence
  PR001763 HFWR1 Chothia, PR001830 HFWR1 Chothia
EVQLLESGGGLVQPGGSLRLSCTAS

SEQ ID NO: 8 - protein, 25 aa, Artificial Sequence
  PR001764 HFWR1 Chothia, PR001768 HFWR1 Chothia, PR001771 HFWR1 Chothia
EVQLLESGGGLVQPGGSLRLSCAAS

SEQ ID NO: 9 - protein, 25 aa, Artificial Sequence
  PR001767 HFWR1 Chothia
EVQLVETGGGLIQPGGSLRLSCAAS

SEQ ID NO: 10 - protein, 25 aa, Artificial Sequence [sequence omitted]

SEQ ID NO: 11 - protein, 25 aa, Artificial Sequence
  PR001780 HFWR1 Chothia
EVQLLESGGGLIQPGGSLRLSCAAS

SEQ ID NO: 12 - protein, 25 aa, Artificial Sequence
  PR002037 HFWR1 Chothia, PR002410 HFWR1 Chothia
QVQLVQSGAEVKKPGSSMRVSCKAS

SEQ ID NO: 13 - protein, 7 aa, Artificial Sequence
  PR000157 HCDR1 Chothia
GYTFTSY

SEQ ID NO: 14 - protein, 7 aa, Artificial Sequence
  PR000448 HCDR1 Chothia, PR000628 HCDR1 Chothia
GGSFSGY

SEQ ID NO: 15 - protein, 7 aa, Artificial Sequence
  PR000483 HCDR1 Chothia
GYSFSTY

SEQ ID NO: 16 - protein, 7 aa, Artificial Sequence
  PR001476 HCDR1 Chothia, PR002408 HCDR1 Chothia
GFTFRSF

SEQ ID NO: 17 - protein, 7 aa, Artificial Sequence
  PR001758 HCDR1 Chothia
GFTFSRY

SEQ ID NO: 18 - protein, 7 aa, Artificial Sequence
  PR001760 HCDR1 Chothia, PR001763 HCDR1 Chothia, PR001768 HCDR1 Chothia
GFTFSNY

SEQ ID NO: 19 - protein, 7 aa, Artificial Sequence
  PR001764 HCDR1 Chothia, PR001781 HCDR1 Chothia, PR001833 HCDR1 Chothia
GFTFSSY

SEQ ID NO: 20 - protein, 7 aa, Artificial Sequence
  PR001767 HCDR1 Chothia
GFTVSSN

SEQ ID NO: 21 - protein, 7 aa, Artificial Sequence
  PR001774 HCDR1 Chothia, PR001780 HCDR1 Chothia
GFTFSSF

SEQ ID NO: 22 - protein, 7 aa, Artificial Sequence
  PR001836 HCDR1 Chothia
GFIFSNF

SEQ ID NO: 23 - protein, 7 aa, Artificial Sequence
  PR002037 HCDR1 Chothia, PR002410 HCDR1 Chothia
EDTFSSY

SEQ ID NO: 24 - protein, 19 aa, Artificial Sequence
  PR000157 HFWR2 Chothia
WIGWVRQAPGQGLEWIGDI

SEQ ID NO: 25 - protein, 19 aa, Artificial Sequence
  PR000448 HFWR2 Chothia
YWSWIRQPPGKGLEWIGEI

SEQ ID NO: 26 - protein, 19 aa, Artificial Sequence
  PR000483 HFWR2 Chothia
WISWVRQMPGKGLEWMGKI

SEQ ID NO: 27 - protein, 19 aa, Artificial Sequence
  PR000628 HFWR2 Chothia
YWSWIRQSPEKGLEWIGEI

SEQ ID NO: 28 - protein, 19 aa, Artificial Sequence
  PR001476 HFWR2 Chothia, PR002408 HFWR2 Chothia
GMHWVRQAPGKGLEWVAVI

SEQ ID NO: 29 - protein, 19 aa, Artificial Sequence
  PR001758 HFWR2 Chothia, PR001760 HFWR2 Chothia, PR001781 HFWR2 Chothia
AMTWVRQAPEKGLEWVSSI

SEQ ID NO: 30 - protein, 19 aa, Artificial Sequence
  PR001763 HFWR2 Chothia, PR001830 HFWR2 Chothia, PR001833 HFWR2 Chothia
AMSWVRQAPEKGLEWVSSI

SEQ ID NO: 31 - protein, 19 aa, Artificial Sequence
  PR001764 HFWR2 Chothia
AMSWVRQAPEKGLEWVSAI

SEQ ID NO: 32 - protein, 19 aa, Artificial Sequence
  PR001767 HFWR2 Chothia
YMSWVRQAPGKGLEWVSVI

SEQ ID NO: 33 - protein, 19 aa, Artificial Sequence
  PR001768 HFWR2 Chothia
AMTWVRQAPGKGLEWVSSI

SEQ ID NO: 34 - protein, 19 aa, Artificial Sequence
  PR001771 HFWR2 Chothia
AMTWVRQPPGKGLEWVSSI

SEQ ID NO: 35 - protein, 19 aa, Artificial Sequence
  PR001774 HFWR2 Chothia
AMTWVRQAPEKGLEWVSTI

SEQ ID NO: 36 - protein, 19 aa, Artificial Sequence
  PR001780 HFWR2 Chothia
AMTWVRQAPGKGLEWVSTI

SEQ ID NO: 37 - protein, 19 aa, Artificial Sequence
  PR001836 HFWR2 Chothia
AMTWVRQPPEKGLKWVSSI

SEQ ID NO: 38 - protein, 19 aa, Artificial Sequence
  PR001838 HFWR2 Chothia, PR004469 HFWR2 Chothia
AMSWFRQPPETGLKWVSSI

SEQ ID NO: 39 - protein, 19 aa, Artificial Sequence
  PR001840 HFWR2 Chothia
WMHWVRQAPGKGLVWVSRI

SEQ ID NO: 40 - protein, 19 aa, Artificial Sequence
  PR001842 HFWR2 Chothia
AMSWGRQAPGKGLEWVSAI

SEQ ID NO: 41 - protein, 19 aa, Artificial Sequence
  PR002037 HFWR2 Chothia, PR002410 HFWR2 Chothia
AISWVRQAPGQGLEWMGGT

SEQ ID NO: 42 - protein, 6 aa, Artificial Sequence
  PR000157 HCDR2 Chothia
YPGGGY

SEQ ID NO: 43 - protein, 5 aa, Artificial Sequence
  PR000448 HCDR2 Chothia
QHSGS

SEQ ID NO: 44 - protein, 6 aa, Artificial Sequence
  PR000483 HCDR2 Chothia
YPGDSY

SEQ ID NO: 45 - protein, 5 aa, Artificial Sequence
  PR000628 HCDR2 Chothia
NHGGY

SEQ ID NO: 46 - protein, 6 aa, Artificial Sequence
  PR001476 HCDR2 Chothia
SYDGSN

SEQ ID NO: 47 - protein, 6 aa, Artificial Sequence
  PR001758 HCDR2 Chothia
SGSGDD

SEQ ID NO: 48 - protein, 6 aa, Artificial Sequence
  PR001760 HCDR2 Chothia
SGSGVS

SEQ ID NO: 49 - protein, 6 aa, Artificial Sequence
  PR001763 HCDR2 Chothia, PR001771 HCDR2 Chothia, PR001830 HCDR2 Chothia
SGSGGS

SEQ ID NO: 50 - protein, 6 aa, Artificial Sequence
  PR001764 HCDR2 Chothia
SGGGGS

SEQ ID NO: 51 - protein, 5 aa, Artificial Sequence
  PR001767 HCDR2 Chothia
YSDGS

SEQ ID NO: 52 - protein, 6 aa, Artificial Sequence
  PR001768 HCDR2 Chothia
SGSGDS

SEQ ID NO: 53 - protein, 6 aa, Artificial Sequence
  PR001774 HCDR2 Chothia
SGSGDT

SEQ ID NO: 54 - protein, 6 aa, Artificial Sequence
  PR001780 HCDR2 Chothia
SGSGDN

SEQ ID NO: 55 - protein, 6 aa, Artificial Sequence
  PR001781 HCDR2 Chothia
SGSGGN

SEQ ID NO: 56 - protein, 6 aa, Artificial Sequence
  PR001836 HCDR2 Chothia
NGSGFN

SEQ ID NO: 57 - protein, 6 aa, Artificial Sequence
  PR001838 HCDR2 Chothia
DGSGGD

SEQ ID NO: 58 - protein, 6 aa, Artificial Sequence
  PR001840 HCDR2 Chothia
NSDGSS

SEQ ID NO: 59 - protein, 6 aa, Artificial Sequence
  PR002037 HCDR2 Chothia, PR002410 HCDR2 Chothia
APIFGT

SEQ ID NO: 60 - protein, 6 aa, Artificial Sequence
  PR002408 HCDR2 Chothia
SYDASN

SEQ ID NO: 61 - protein, 6 aa, Artificial Sequence
  PR004469 HCDR2 Chothia, PR007381 HCDR2 Chothia
DASGGD

SEQ ID NO: 62 - protein, 41 aa, Artificial Sequence
  PR000157 HFWR3 Chothia
TNYNEKFKGRVTITRDTSTSTAYLELSSLRSEDTAVYYCAR

SEQ ID NO: 63 - protein, 41 aa, Artificial Sequence
  PR000448 HFWR3 Chothia
TDSNPSLKGRVTFSVDTSKNQFSLKLNSVTAADTAVYYCAR

SEQ ID NO: 64 - protein, 41 aa, Artificial Sequence
  PR000483 HFWR3 Chothia
TNYSPSFQGQVTISADKSISTAYLQWSSLKASDTAMYYCAR

SEQ ID NO: 65 - protein, 41 aa, Artificial Sequence
  PR000628 HFWR3 Chothia
VTYNPSLESRVTISVDTSKNQFSLKLSSVTAADTAVYYCAR

SEQ ID NO: 66 - protein, 41 aa, Artificial Sequence
  PR001476 HFWR3 Chothia, PR002408 HFWR3 Chothia
EYYADSVKGRFIISRDNSKDTLYLQMNSLRAGDTAVYYCAK

SEQ ID NO: 67 - protein, 41 aa, Artificial Sequence
  PR001758 HFWR3 Chothia
TYYGDSVKGRFTISRDNSQNTVYLQMNSLRAEDTAVYFCAK

SEQ ID NO: 68 - protein, 41 aa, Artificial Sequence
  PR001760 HFWR3 Chothia
TYYADSVKGRFTISRDNSKNTLYLQMTRLTAEDTAVYFCAK

SEQ ID NO: 69 - protein, 41 aa, Artificial Sequence
  PR001763 HFWR3 Chothia
TFYADSVKGRFTISRDNSKNTLYLQMNRLTAEDTAVYYCAK

SEQ ID NO: 70 - protein, 41 aa, Artificial Sequence
  PR001764 HFWR3 Chothia
TYYADSVKGRFTISRDNSKNTLYLQMDSLKAEDTAVYYCAK

SEQ ID NO: 71 - protein, 41 aa, Artificial Sequence
  PR001767 HFWR3 Chothia
TYYADSVKGRFTISRDNSKNTLYLQMNSLRAEDTAVYYCAR

SEQ ID NO: 72 - protein, 41 aa, Artificial Sequence
  PR001768 HFWR3 Chothia, PR001771 HFWR3 Chothia, PR001781 HFWR3 Chothia
TYYADSVKGRFTISRDNSKNTLYLQMNSLRAEDTAVYYCAK

SEQ ID NO: 73 - protein, 41 aa, Artificial Sequence
  PR001774 HFWR3 Chothia
TYYADSVKGRFTISRDSSKNTLYLQMNSLRAEDSAVYFCAK

SEQ ID NO: 74 - protein, 41 aa, Artificial Sequence
  PR001780 HFWR3 Chothia
TYYADSVKGRFTISRDNSKNTLYLQMNSLRAEDTAVYFCAK

SEQ ID NO: 75 - protein, 41 aa, Artificial Sequence
  PR001830 HFWR3 Chothia, PR001833 HFWR3 Chothia
TFYADSVKGRFTISRDNSKNTLYLQMNSLRAEDTAVYFCAK

SEQ ID NO: 76 - protein, 41 aa, Artificial Sequence
  PR001836 HFWR3 Chothia
TYYTDSVKGRFTISRDNSRNTLYLQMNRLTAEDTAVYFCAK

SEQ ID NO: 77 - protein, 41 aa, Artificial Sequence
  PR001840 HFWR3 Chothia
TSYADSVQGRFTISRDNAKNTLYLQMNSLRAEDTAVYYCVR

SEQ ID NO: 78 - protein, 41 aa, Artificial Sequence
  PR001842 HFWR3 Chothia
TYYADSVKGRFTISRDNSKNTLYLHMNSLRAEDTAVYYCAK

SEQ ID NO: 79 - protein, 41 aa, Artificial Sequence
  PR002037 HFWR3 Chothia, PR002410 HFWR3 Chothia
TNYAQKFQGRVTITADKSTSTAYMELSSLRSEDTAVYYCAR

SEQ ID NO: 80 - protein, 12 aa, Artificial Sequence
  PR000157 HCDR3 Chothia
LAGSSYRGAMDS

SEQ ID NO: 81 - protein, 7 aa, Artificial Sequence
  PR000448 HCDR3 Chothia
LTGPFDY

SEQ ID NO: 82 - protein, 7 aa, Artificial Sequence
  PR000483 HCDR3 Chothia
GYGIFDY

SEQ ID NO: 83 - protein, 13 aa, Artificial Sequence
  PR000628 HCDR3 Chothia
DYGPGNYDWYFDL

SEQ ID NO: 84 - protein, 10 aa, Artificial Sequence
  PR001476 HCDR3 Chothia, PR002408 HCDR3 Chothia
GGGLRWYFAY

SEQ ID NO: 85 - protein, 15 aa, Artificial Sequence
  PR001758 HCDR3 Chothia
EKAGTTGDYYYNVDV

SEQ ID NO: 86 - protein, 15 aa, Artificial Sequence
  PR001760 HCDR3 Chothia, PR001830 HCDR3 Chothia, PR001836 HCDR3 Chothia
EGSSETDDHYYNVDV

SEQ ID NO: 87 - protein, 15 aa, Artificial Sequence
  PR001763 HCDR3 Chothia
EGSNGTDDYHYDIDV

SEQ ID NO: 88 - protein, 15 aa, Artificial Sequence
  PR001764 HCDR3 Chothia
EGTTETDDYHYNMDV

SEQ ID NO: 89 - protein, 18 aa, Artificial Sequence
  PR001767 HCDR3 Chothia
DRYYGSGNYPTAYYGMDV

SEQ ID NO: 90 - protein, 15 aa, Artificial Sequence
  PR001768 HCDR3 Chothia, PR001771 HCDR3 Chothia
EGTGTTSDYYYNVDV

SEQ ID NO: 91 - protein, 15 aa, Artificial Sequence
  PR001774 HCDR3 Chothia
EATAMASDYYYGVDV

SEQ ID NO: 92 - protein, 15 aa, Artificial Sequence
  PR001780 HCDR3 Chothia
EDTAVASDYYYNIDV

SEQ ID NO: 93 - protein, 15 aa, Artificial Sequence
  PR001781 HCDR3 Chothia
ERTGTTGDYYYNVDV

SEQ ID NO: 94 - protein, 15 aa, Artificial Sequence
  PR001833 HCDR3 Chothia
EGATETDDYHFNTDV

SEQ ID NO: 95 - protein, 15 aa, Artificial Sequence
  PR001838 HCDR3 Chothia, PR004469 HCDR3 Chothia, PR007381 HCDR3 Chothia
EGSHGTDDSHYDVDV

SEQ ID NO: 96 - protein, 14 aa, Artificial Sequence
  PR001840 HCDR3 Chothia
KGSSSYYHYSIEDD

SEQ ID NO: 97 - protein, 15 aa, Artificial Sequence
  PR001842 HCDR3 Chothia
EKVATTGDYYYDMDV

SEQ ID NO: 98 - protein, 7 aa, Artificial Sequence
  PR002037 HCDR3 Chothia, PR002410 HCDR3 Chothia
GGPYFDY

SEQ ID NO: 99 - protein, 11 aa, Artificial Sequence
  PR000157 HFWR4 Chothia, PR000448 HFWR4 Chothia, PR000483 HFWR4 Chothia
WGQGTLVTVSS

SEQ ID NO: 100 - protein, 11 aa, Artificial Sequence
  PR000628 HFWR4 Chothia
WGRGTLVTVSS

SEQ ID NO: 101 - protein, 11 aa, Artificial Sequence
  PR001758 HFWR4 Chothia, PR001760 HFWR4 Chothia, PR001763 HFWR4 Chothia
WGQGTTVTVSS

SEQ ID NO: 102 - protein, 11 aa, Artificial Sequence
  PR001767 HFWR4 Chothia
RGQGTTVTVSS

SEQ ID NO: 103 - protein, 23 aa, Artificial Sequence
  PR000157 LFWR1 Chothia
DIQMTQSPSSLSASVGDRVTITC

SEQ ID NO: 104 - protein, 23 aa, Artificial Sequence
  PR000448 LFWR1 Chothia, PR001476 LFWR1 Chothia, PR002408 LFWR1 Chothia
EIVMTQSPATLSVSPGERATLSC

SEQ ID NO: 105 - protein, 22 aa, Artificial Sequence
  PR000483 LFWR1 Chothia
SYELTQPPSVSVSPGQTASITC

SEQ ID NO: 106 - protein, 23 aa, Artificial Sequence
  PR000628 LFWR1 Chothia
EIVLTQSPATLSLSPGERATLSC

SEQ ID NO: 107 - protein, 23 aa, Artificial Sequence
  PR002037 LFWR1 Chothia, PR002410 LFWR1 Chothia
EIVMTQSPASLSVSPGERATLSC

SEQ ID NO: 108 - protein, 11 aa, Artificial Sequence
  PR000157 LCDR1 Chothia
KASQGFNKYVA

SEQ ID NO: 109 - protein, 11 aa, Artificial Sequence
  PR000448 LCDR1 Chothia
RASQSISSILA

SEQ ID NO: 110 - protein, 11 aa, Artificial Sequence
  PR000483 LCDR1 Chothia
SGDNIGDQYAH

SEQ ID NO: 111 - protein, 11 aa, Artificial Sequence
  PR000628 LCDR1 Chothia
RASQSVSSYLA

SEQ ID NO: 112 - protein, 11 aa, Artificial Sequence
  PR001476 LCDR1 Chothia, PR002408 LCDR1 Chothia
RASQSISSNLG

SEQ ID NO: 113 - protein, 11 aa, Artificial Sequence
  PR002037 LCDR1 Chothia, PR002410 LCDR1 Chothia
RASQSVSSNLA

SEQ ID NO: 114 - protein, 15 aa, Artificial Sequence
  PR000157 LFWR2 Chothia
WYQQKPGKAPKLLIY

SEQ ID NO: 115 - protein, 15 aa, Artificial Sequence
  PR000448 LFWR2 Chothia, PR000628 LFWR2 Chothia, PR001476 LFWR2 Chothia
WYQQKPGQAPRLLIY

SEQ ID NO: 116 - protein, 15 aa, Artificial Sequence
  PR000483 LFWR2 Chothia
WYQQKPGQSPVLVIY

SEQ ID NO: 117 - protein, 7 aa, Artificial Sequence
  PR000157 LCDR2 Chothia
YTSTLQP

SEQ ID NO: 118 - protein, 7 aa, Artificial Sequence
  PR000448 LCDR2 Chothia, PR001476 LCDR2 Chothia, PR002037 LCDR2 Chothia
GASTRAT

SEQ ID NO: 119 - protein, 7 aa, Artificial Sequence
  PR000483 LCDR2 Chothia
QDKNRPS

SEQ ID NO: 120 - protein, 7 aa, Artificial Sequence
  PR000628 LCDR2 Chothia
DASNRAT

SEQ ID NO: 121 - protein, 32 aa, Artificial Sequence
  PR000157 LFWR3 Chothia
GVPSRFSGSGSGRDYTLTISSLQPEDFATYYC

SEQ ID NO: 122 - protein, 32 aa, Artificial Sequence
  PR000448 LFWR3 Chothia, PR001476 LFWR3 Chothia, PR002408 LFWR3 Chothia
GIPARFSGSGSGTEFTLTISSLQSEDFAVYYC

SEQ ID NO: 123 - protein, 32 aa, Artificial Sequence
  PR000483 LFWR3 Chothia
GIPERFSGSNSGNTATLTISGTQAMDEADYYC

SEQ ID NO: 124 - protein, 32 aa, Artificial Sequence
  PR000628 LFWR3 Chothia
GIPARFSGSGSGTDFTLTISSLEPEDFAVYYC

SEQ ID NO: 125 - protein, 32 aa, Artificial Sequence
  PR002037 LFWR3 Chothia
GIPARVSGGGSGTEFTLTISSLQSEDFAVYCC

SEQ ID NO: 126 - protein, 32 aa, Artificial Sequence
  PR002410 LFWR3 Chothia
GIPARVSGGGSGTEFTLTISSLQSEDFAVYYC

SEQ ID NO: 127 - protein, 9 aa, Artificial Sequence
  PR000157 LCDR3 Chothia
LQYGDLLYA

SEQ ID NO: 128 - protein, 9 aa, Artificial Sequence
  PR000448 LCDR3 Chothia
QQYYNWPLT

SEQ ID NO: 129 - protein, 11 aa, Artificial Sequence
  PR000483 LCDR3 Chothia
ATYTGFGSLAV

SEQ ID NO: 130 - protein, 11 aa, Artificial Sequence
  PR000628 LCDR3 Chothia
QQRSNWPPALT

SEQ ID NO: 131 - protein, 10 aa, Artificial Sequence
  PR001476 LCDR3 Chothia
QQYNSWPPLT

SEQ ID NO: 132 - protein, 9 aa, Artificial Sequence
  PR002037 LCDR3 Chothia, PR002410 LCDR3 Chothia
QQYKNWPFT

SEQ ID NO: 133 - protein, 10 aa, Artificial Sequence
  PR002408 LCDR3 Chothia
QQYQSWPPLT

SEQ ID NO: 134 - protein, 10 aa, Artificial Sequence
  PR000157 LFWR4 Chothia
FGQGTKVEIK

SEQ ID NO: 135 - protein, 10 aa, Artificial Sequence
  PR000448 LFWR4 Chothia, PR000628 LFWR4 Chothia, PR001476 LFWR4 Chothia
FGGGTKVEIK

SEQ ID NO: 136 - protein, 10 aa, Artificial Sequence
  PR000483 LFWR4 Chothia
FGGGTKLTVL

SEQ ID NO: 137 - protein, 10 aa, Artificial Sequence
  PR002037 LFWR4 Chothia, PR002410 LFWR4 Chothia
FGPGTKLEIK

SEQ ID NO: 138 - protein, 121 aa, Artificial Sequence
  PR000157 VH
EVQLVQSGAEVKKPGASVKVSCKASGYTFTSYWIGWVRQAPGQGLEWIGDIYPGGGYTNYNEKFKGRVTITRDTSTSTAYLELSSLRSEDTAVYYCARLAGSSYRGAMDSWGQGTLVTVSS

SEQ ID NO: 139 - protein, 115 aa, Artificial Sequence
  PR000448 VH
QVQLQQWGAGLLKPSETLSLTCAVYGGSFSGYYWSWIRQPPGKGLEWIGEIQHSGSTDSNPSLKGRVTFSVDTSKNQFSLKLNSVTAADTAVYYCARLTGPFDYWGQGTLVTVSS

SEQ ID NO: 140 - protein, 116 aa, Artificial Sequence
  PR000483 VH
EVQLVQSGAEVKKPGESLRISCKGSGYSFSTYWISWVRQMPGKGLEWMGKIYPGDSYTNYSPSFQGQVTISADKSISTAYLQWSSLKASDTAMYYCARGYGIFDYWGQGTLVTVSS

SEQ ID NO: 141 - protein, 121 aa, Artificial Sequence [sequence omitted]

SEQ ID NO: 142 - protein, 119 aa, Artificial Sequence
  PR001476 VH
QVQLVESGGGVVQPGRSLRLSCAASGFTFRSFGMHWVRQAPGKGLEWVAVISYDGSNEYYADSVKGRFIISRDNSKDTLYLQMNSLRAGDTAVYYCAKGGGLRWYFAYWGQGTLVTVSS

SEQ ID NO: 143 - protein, 124 aa, Artificial Sequence
  PR001758 VH
EVQLLESGGGLVQLGGSLRLSCAASGFTFSRYAMTWVRQAPEKGLEWVSSISGSGDDTYYGDSVKGRFTISRDNSQNTVYLQMNSLRAEDTAVYFCAKEKAGTTGDYYYNVDVWGQGTTVTVSS

SEQ ID NO: 144 - protein, 124 aa, Artificial Sequence
  PR001760 VH
EVQLVESGGGVVQPGGSLRLSCAASGFTFSNYAMTWVRQAPEKGLEWVSSISGSGVSTYYADSVKGRFTISRDNSKNTLYLQMTRLTAEDTAVYFCAKEGSSETDDHYYNVDVWGQGTTVTVSS

SEQ ID NO: 145 - protein, 124 aa, Artificial Sequence
  PR001763 VH
EVQLLESGGGLVQPGGSLRLSCTASGFTFSNYAMSWVRQAPEKGLEWVSSISGSGGSTFYADSVKGRFTISRDNSKNTLYLQMNRLTAEDTAVYYCAKEGSNGTDDYHYDIDVWGQGTTVTVSS

SEQ ID NO: 146 - protein, 124 aa, Artificial Sequence
  PR001764 VH
EVQLLESGGGLVQPGGSLRLSCAASGFTFSSYAMSWVRQAPEKGLEWVSAISGGGGSTYYADSVKGRFTISRDNSKNTLYLQMDSLKAEDTAVYYCAKEGTTETDDYHYNMDVWGQGTTVTVSS

SEQ ID NO: 147 - protein, 126 aa, Artificial Sequence
  PR001767 VH
EVQLVETGGGLIQPGGSLRLSCAASGFTVSSNYMSWVRQAPGKGLEWVSVIYSDGSTYYADSVKGRFTISRDNSKNTLYLQMNSLRAEDTAVYYCARDRYYGSGNYPTAYYGMDVRGQGTTVTVSS

SEQ ID NO: 148 - protein, 124 aa, Artificial Sequence
  PR001768 VH
EVQLLESGGGLVQPGGSLRLSCAASGFTFSNYAMTWVRQAPGKGLEWVSSISGSGDSTYYADSVKGRFTISRDNSKNTLYLQMNSLRAEDTAVYYCAKEGTGTTSDYYYNVDVWGQGTTVTVSS

SEQ ID NO: 149 - protein, 124 aa, Artificial Sequence
  PR001771 VH
EVQLLESGGGLVQPGGSLRLSCAASGFTFSNYAMTWVRQPPGKGLEWVSSISGSGGSTYYADSVKGRFTISRDNSKNTLYLQMNSLRAEDTAVYYCAKEGTGTTSDYYYNVDVWGQGTTVTVSS

SEQ ID NO: 150 - protein, 124 aa, Artificial Sequence
  PR001774 VH
EVQLVESGGGLVQPGGSLRLSCAASGFTFSSFAMTWVRQAPEKGLEWVSTISGSGDTTYYADSVKGRFTISRDSSKNTLYLQMNSLRAEDSAVYFCAKEATAMASDYYYGVDVWGQGTTVTVSS

SEQ ID NO: 151 - protein, 124 aa, Artificial Sequence
  PR001780 VH
EVQLLESGGGLIQPGGSLRLSCAASGFTFSSFAMTWVRQAPGKGLEWVSTISGSGDNTYYADSVKGRFTISRDNSKNTLYLQMNSLRAEDTAVYFCAKEDTAVASDYYYNIDVWGQGTTVTVSS

SEQ ID NO: 152 - protein, 124 aa, Artificial Sequence
  PR001781 VH
EVQLLESGGGLVQLGGSLRLSCAASGFTFSSYAMTWVRQAPEKGLEWVSSISGSGGNTYYADSVKGRFTISRDNSKNTLYLQMNSLRAEDTAVYYCAKERTGTTGDYYYNVDVWGQGTTVTVSS

SEQ ID NO: 153 - protein, 124 aa, Artificial Sequence
  PR001830 VH
EVQLLESGGGLVQPGGSLRLSCTASGFTFSNYAMSWVRQAPEKGLEWVSSISGSGGSTFYADSVKGRFTISRDNSKNTLYLQMNSLRAEDTAVYFCAKEGSSETDDHYYNVDVWGQGTTVTVSS

SEQ ID NO: 154 - protein, 124 aa, Artificial Sequence
  PR001833 VH
EVQLLESGGGLVQPGGSLRLSCAASGFTFSSYAMSWVRQAPEKGLEWVSSISGSGGSTFYADSVKGRFTISRDNSKNTLYLQMNSLRAEDTAVYFCAKEGATETDDYHFNTDVWGQGTTVTVSS

SEQ ID NO: 155 - protein, 124 aa, Artificial Sequence
  PR001836 VH
EVQLLESGGGLVQPGGSLRLSCAASGFIFSNFAMTWVRQPPEKGLKWVSSINGSGFNTYYTDSVKGRFTISRDNSRNTLYLQMNRLTAEDTAVYFCAKEGSSETDDHYYNVDVWGQGTTVTVSS

SEQ ID NO: 156 - protein, 124 aa, Artificial Sequence
  PR001838 VH
EVQLLESGGGLVQPGGSLRLSCAASGFTFSNYAMSWFRQPPETGLKWVSSIDGSGGDTYYADSVKGRFTISRDNSKNTLYLQMNSLRAEDTAVYYCAKEGSHGTDDSHYDVDVWGQGTTVTVSS

SEQ ID NO: 157 - protein, 123 aa, Artificial Sequence
  PR001840 VH
EVQLVESGGGLVQPGGSLRLSCAASGFTFSSYWMHWVRQAPGKGLVWVSRINSDGSSTSYADSVQGRFTISRDNAKNTLYLQMNSLRAEDTAVYYCVRKGSSSYYHYSIEDDWGQGTLVTVSS

SEQ ID NO: 158 - protein, 124 aa, Artificial Sequence
  PR001842 VH
EVQLLESGGGLVQPGGSLRLSCAASGFTFSSYAMSWGRQAPGKGLEWVSAISGSGGSTYYADSVKGRFTISRDNSKNTLYLHMNSLRAEDTAVYYCAKEKVATTGDYYYDMDVWGQGTTVTVSS

SEQ ID NO: 159 - protein, 116 aa, Artificial Sequence
  PR002037 VH, PR002410 VH
QVQLVQSGAEVKKPGSSMRVSCKASEDTFSSYAISWVRQAPGQGLEWMGGTAPIFGTTNYAQKFQGRVTITADKSTSTAYMELSSLRSEDTAVYYCARGGPYFDYWGQGTLVTVSS

SEQ ID NO: 160 - protein, 119 aa, Artificial Sequence
  PR002408 VH
QVQLVESGGGVVQPGRSLRLSCAASGFTFRSFGMHWVRQAPGKGLEWVAVISYDASNEYYADSVKGRFIISRDNSKDTLYLQMNSLRAGDTAVYYCAKGGGLRWYFAYWGQGTLVTVSS

SEQ ID NO: 161 - protein, 124 aa, Artificial Sequence
  PR004469 VH
EVQLLESGGGLVQPGGSLRLSCAASGFTFSNYAMSWFRQPPETGLKWVSSIDASGGDTYYADSVKGRFTISRDNSKNTLYLQMNSLRAEDTAVYYCAKEGSHGTDDSHYDVDVWGQGTTVTVSS

SEQ ID NO: 162 - protein, 107 aa, Artificial Sequence
  PR000157 VL
DIQMTQSPSSLSASVGDRVTITCKASQGFNKYVAWYQQKPGKAPKLLIYYTSTLQPGVPSRFSGSGSGRDYTLTISSLQPEDFATYYCLQYGDLLYAFGQGTKVEIK

SEQ ID NO: 163 - protein, 107 aa, Artificial Sequence
  PR000448 VL
EIVMTQSPATLSVSPGERATLSCRASQSISSILAWYQQKPGQAPRLLIYGASTRATGIPARFSGSGSGTEFTLTISSLQSEDFAVYYCQQYYNWPLTFGGGTKVEIK

SEQ ID NO: 164 - protein, 108 aa, Artificial Sequence
  PR000483 VL
SYELTQPPSVSVSPGQTASITCSGDNIGDQYAHWYQQKPGQSPVLVIYQDKNRPSGIPERFSGSNSGNTATLTISGTQAMDEADYYCATYTGFGSLAVFGGGTKLTVL

SEQ ID NO: 165 - protein, 109 aa, Artificial Sequence [sequence omitted]

SEQ ID NO: 166 - protein, 108 aa, Artificial Sequence
  PR001476 VL
EIVMTQSPATLSVSPGERATLSCRASQSISSNLGWYQQKPGQAPRLLIYGASTRATGIPARFSGSGSGTEFTLTISSLQSEDFAVYYCQQYNSWPPLTFGGGTKVEIK

SEQ ID NO: 167 - protein, 107 aa, Artificial Sequence
  PR002037 VL
EIVMTQSPASLSVSPGERATLSCRASQSVSSNLAWYQQKPGQAPRLLIYGASTRATGIPARVSGGGSGTEFTLTISSLQSEDFAVYCCQQYKNWPFTFGPGTKLEIK

SEQ ID NO: 168 - protein, 108 aa, Artificial Sequence
  PR002408 VL
EIVMTQSPATLSVSPGERATLSCRASQSISSNLGWYQQKPGQAPRLLIYGASTRATGIPARFSGSGSGTEFTLTISSLQSEDFAVYYCQQYQSWPPLTFGGGTKVEIK

SEQ ID NO: 169 - protein, 107 aa, Artificial Sequence
  PR002410 VL
EIVMTQSPASLSVSPGERATLSCRASQSVSSNLAWYQQKPGQAPRLLIYGASTRATGIPARVSGGGSGTEFTLTISSLQSEDFAVYYCQQYKNWPFTFGPGTKLEIK

SEQ ID NO: 170 - protein, 451 aa, Artificial Sequence
  PR000157 HC
EVQLVQSGAEVKKPGASVKVSCKASGYTFTSYWIGWVRQAPGQGLEWIGDIYPGGGYTNYNEKFKGRVTITRDTSTSTAYLELSSLRSEDTAVYYCARLAGSSYRGAMDSWGQGTLVTVSSASTKGPSVFPLAPSSKSTSGGTAALGCLVKDYFPEPVTVSWNSGALTSGVHTFPAVLQSSGLYSLSSVVTVPSSSLGTQTYICNVNHKPSNTKVDKKVEPKSCDKTHTCPPCPAPELLGGPSVFLFPPKPKDTLMISRTPEVTCVVVDVSHEDPEVKFNWYVDGVEVHNAKTKPREEQYNSTYRVVSVLTVLHQDWLNGKEYKCKVSNKALPAPIEKTISKAKGQPREPQVYTLPPSREEMTKNQVSLTCLVKGFYPSDIAVEWESNGQPENNYKTTPPVLDSDGSFFLYSKLTVDKSRWQQGNVFSCSVMHEALHNHYTQKSLSLSPGK

SEQ ID NO: 171 - protein, 442 aa, Artificial Sequence
  PR000448 HC
QVQLQQWGAGLLKPSETLSLTCAVYGGSFSGYYWSWIRQPPGKGLEWIGEIQHSGSTDSNPSLKGRVTFSVDTSKNQFSLKLNSVTAADTAVYYCARLTGPFDYWGQGTLVTVSSASTKGPSVFPLAPCSRSTSESTAALGCLVKDYFPEPVTVSWNSGALTSGVHTFPAVLQSSGLYSLSSVVTVPSSSLGTKTYTCNVDHKPSNTKVDKRVESKYGPPCPPCPAPEFLGGPSVFLFPPKPKDTLMISRTPEVTCVVVDVSQEDPEVQFNWYVDGVEVHNAKTKPREEQFNSTYRVVSVLTVLHQDWLNGKEYKCKVSNKGLPSSIEKTISKAKGQPREPQVYTLPPSQEEMTKNQVSLTCLVKGFYPSDIAVEWESNGQPENNYKTTPPVLDSDGSFFLYSRLTVDKSRWQEGNVFSCSVMHEALHNHYTQKSLSLSLGK

SEQ ID NO: 172 - protein, 442 aa, Artificial Sequence
  PR000483 HC
EVQLVQSGAEVKKPGESLRISCKGSGYSFSTYWISWVRQMPGKGLEWMGKIYPGDSYTNYSPSFQGQVTISADKSISTAYLQWSSLKASDTAMYYCARGYGIFDYWGQGTLVTVSSASTKGPSVFPLAPCSRSTSESTAALGCLVKDYFPEPVTVSWNSGALTSGVHTFPAVLQSSGLYSLSSVVTVPSSNFGTQTYTCNVDHKPSNTKVDKTVERKCCVECPPCPAPPVAGPSVFLFPPKPKDTLMISRTPEVTCVVVDVSHEDPEVQFNWYVDGVEVHNAKTKPREEQFNSTFRVVSVLTVVHQDWLNGKEYKCKVSNKGLPAPIEKTISKTKGQPREPQVYTLPPSREEMTKNQVSLTCLVKGFYPSDIAVEWESNGQPENNYKTTPPMLDSDGSFFLYSKLTVDKSRWQQGNVFSCSVMHEALHNHYTQKSLSLSPGK

SEQ ID NO: 173 - protein, 448 aa, Artificial Sequence
  PR000628 HC
QVQLQQWGAGLLKPSETLSLTCAVYGGSFSGYYWSWIRQSPEKGLEWIGEINHGGYVTYNPSLESRVTISVDTSKNQFSLKLSSVTAADTAVYYCARDYGPGNYDWYFDLWGRGTLVTVSSASTKGPSVFPLAPCSRSTSESTAALGCLVKDYFPEPVTVSWNSGALTSGVHTFPAVLQSSGLYSLSSVVTVPSSSLGTKTYTCNVDHKPSNTKVDKRVESKYGPPCPPCPAPEFLGGPSVFLFPPKPKDTLMISRTPEVTCVVVDVSQEDPEVQFNWYVDGVEVHNAKTKPREEQFNSTYRVVSVLTVLHQDWLNGKEYKCKVSNKGLPSSIEKTISKAKGQPREPQVYTLPPSQEEMTKNQVSLTCLVKGFYPSDIAVEWESNGQPENNYKTTPPVLDSDGSFFLYSRLTVDKSRWQEGNVFSCSVMHEALHNHYTQKSLSLSLGK

SEQ ID NO: 174 - protein, 449 aa, Artificial Sequence
  PR001476 HC
QVQLVESGGGVVQPGRSLRLSCAASGFTFRSFGMHWVRQAPGKGLEWVAVISYDGSNEYYADSVKGRFIISRDNSKDTLYLQMNSLRAGDTAVYYCAKGGGLRWYFAYWGQGTLVTVSSASTKGPSVFPLAPSSKSTSGGTAALGCLVKDYFPEPVTVSWNSGALTSGVHTFPAVLQSSGLYSLSSVVTVPSSSLGTQTYICNVNHKPSNTKVDKKVEPKSCDKTHTCPPCPAPELLGGPSVFLFPPKPKDTLMISRTPEVTCVVVDVSHEDPEVKFNWYVDGVEVHNAKTKPREEQYNSTYRVVSVLTVLHQDWLNGKEYKCKVSNKALPAPIEKTISKAKGQPREPQVYTLPPSREEMTKNQVSLTCLVKGFYPSDIAVEWESNGQPENNYKTTPPVLDSDGSFFLYSKLTVDKSRWQQGNVFSCSVMHEALHNHYTQKSLSLSPGK

SEQ ID NO: 175 - protein, 356 aa, Artificial Sequence
  PR001758 HC
EVQLLESGGGLVQLGGSLRLSCAASGFTFSRYAMTWVRQAPEKGLEWVSSISGSGDDTYYGDSVKGRFTISRDNSQNTVYLQMNSLRAEDTAVYFCAKEKAGTTGDYYYNVDVWGQGTTVTVSSEPKSCDKTHTCPPCPAPELLGGPSVFLFPPKPKDTLMISRTPEVTCVVVDVSHEDPEVKFNWYVDGVEVHNAKTKPREEQYNSTYRVVSVLTVLHQDWLNGKEYKCKVSNKALPAPIEKTISKAKGQPREPQVYTLPPSREEMTKNQVSLTCLVKGFYPSDIAVEWESNGQPENNYKTTPPVLDSDGSFFLYSKLTVDKSRWQQGNVFSCSVMHEALHNHYTQKSLSLSPGK

SEQ ID NO: 176 - protein, 356 aa, Artificial Sequence
  PR001760 HC
EVQLVESGGGVVQPGGSLRLSCAASGFTFSNYAMTWVRQAPEKGLEWVSSISGSGVSTYYADSVKGRFTISRDNSKNTLYLQMTRLTAEDTAVYFCAKEGSSETDDHYYNVDVWGQGTTVTVSSEPKSCDKTHTCPPCPAPELLGGPSVFLFPPKPKDTLMISRTPEVTCVVVDVSHEDPEVKFNWYVDGVEVHNAKTKPREEQYNSTYRVVSVLTVLHQDWLNGKEYKCKVSNKALPAPIEKTISKAKGQPREPQVYTLPPSREEMTKNQVSLTCLVKGFYPSDIAVEWESNGQPENNYKTTPPVLDSDGSFFLYSKLTVDKSRWQQGNVFSCSVMHEALHNHYTQKSLSLSPGK

SEQ ID NO: 177 - protein, 356 aa, Artificial Sequence
  PR001763 HC
EVQLLESGGGLVQPGGSLRLSCTASGFTFSNYAMSWVRQAPEKGLEWVSSISGSGGSTFYADSVKGRFTISRDNSKNTLYLQMNRLTAEDTAVYYCAKEGSNGTDDYHYDIDVWGQGTTVTVSSEPKSCDKTHTCPPCPAPELLGGPSVFLFPPKPKDTLMISRTPEVTCVVVDVSHEDPEVKFNWYVDGVEVHNAKTKPREEQYNSTYRVVSVLTVLHQDWLNGKEYKCKVSNKALPAPIEKTISKAKGQPREPQVYTLPPSREEMTKNQVSLTCLVKGFYPSDIAVEWESNGQPENNYKTTPPVLDSDGSFFLYSKLTVDKSRWQQGNVFSCSVMHEALHNHYTQKSLSLSPGK

SEQ ID NO: 178 - protein, 356 aa, Artificial Sequence
  PR001764 HC
EVQLLESGGGLVQPGGSLRLSCAASGFTFSSYAMSWVRQAPEKGLEWVSAISGGGGSTYYADSVKGRFTISRDNSKNTLYLQMDSLKAEDTAVYYCAKEGTTETDDYHYNMDVWGQGTTVTVSSEPKSCDKTHTCPPCPAPELLGGPSVFLFPPKPKDTLMISRTPEVTCVVVDVSHEDPEVKFNWYVDGVEVHNAKTKPREEQYNSTYRVVSVLTVLHQDWLNGKEYKCKVSNKALPAPIEKTISKAKGQPREPQVYTLPPSREEMTKNQVSLTCLVKGFYPSDIAVEWESNGQPENNYKTTPPVLDSDGSFFLYSKLTVDKSRWQQGNVFSCSVMHEALHNHYTQKSLSLSPGK

SEQ ID NO: 179 - protein, 358 aa, Artificial Sequence
  PR001767 HC
EVQLVETGGGLIQPGGSLRLSCAASGFTVSSNYMSWVRQAPGKGLEWVSVIYSDGSTYYADSVKGRFTISRDNSKNTLYLQMNSLRAEDTAVYYCARDRYYGSGNYPTAYYGMDVRGQGTTVTVSSEPKSCDKTHTCPPCPAPELLGGPSVFLFPPKPKDTLMISRTPEVTCVVVDVSHEDPEVKFNWYVDGVEVHNAKTKPREEQYNSTYRVVSVLTVLHQDWLNGKEYKCKVSNKALPAPIEKTISKAKGQPREPQVYTLPPSREEMTKNQVSLTCLVKGFYPSDIAVEWESNGQPENNYKTTPPVLDSDGSFFLYSKLTVDKSRWQQGNVFSCSVMHEALHNHYTQKSLSLSPGK

SEQ ID NO: 180 - protein, 356 aa, Artificial Sequence
  PR001768 HC
EVQLLESGGGLVQPGGSLRLSCAASGFTFSNYAMTWVRQAPGKGLEWVSSISGSGDSTYYADSVKGRFTISRDNSKNTLYLQMNSLRAEDTAVYYCAKEGTGTTSDYYYNVDVWGQGTTVTVSSEPKSCDKTHTCPPCPAPELLGGPSVFLFPPKPKDTLMISRTPEVTCVVVDVSHEDPEVKFNWYVDGVEVHNAKTKPREEQYNSTYRVVSVLTVLHQDWLNGKEYKCKVSNKALPAPIEKTISKAKGQPREPQVYTLPPSREEMTKNQVSLTCLVKGFYPSDIAVEWESNGQPENNYKTTPPVLDSDGSFFLYSKLTVDKSRWQQGNVFSCSVMHEALHNHYTQKSLSLSPGK

SEQ ID NO: 181 - protein, 356 aa, Artificial Sequence
  PR001771 HC
EVQLLESGGGLVQPGGSLRLSCAASGFTFSNYAMTWVRQPPGKGLEWVSSISGSGGSTYYADSVKGRFTISRDNSKNTLYLQMNSLRAEDTAVYYCAKEGTGTTSDYYYNVDVWGQGTTVTVSSEPKSCDKTHTCPPCPAPELLGGPSVFLFPPKPKDTLMISRTPEVTCVVVDVSHEDPEVKFNWYVDGVEVHNAKTKPREEQYNSTYRVVSVLTVLHQDWLNGKEYKCKVSNKALPAPIEKTISKAKGQPREPQVYTLPPSREEMTKNQVSLTCLVKGFYPSDIAVEWESNGQPENNYKTTPPVLDSDGSFFLYSKLTVDKSRWQQGNVFSCSVMHEALHNHYTQKSLSLSPGK

SEQ ID NO: 182 - protein, 356 aa, Artificial Sequence
  PR001774 HC
EVQLVESGGGLVQPGGSLRLSCAASGFTFSSFAMTWVRQAPEKGLEWVSTISGSGDTTYYADSVKGRFTISRDSSKNTLYLQMNSLRAEDSAVYFCAKEATAMASDYYYGVDVWGQGTTVTVSSEPKSCDKTHTCPPCPAPELLGGPSVFLFPPKPKDTLMISRTPEVTCVVVDVSHEDPEVKFNWYVDGVEVHNAKTKPREEQYNSTYRVVSVLTVLHQDWLNGKEYKCKVSNKALPAPIEKTISKAKGQPREPQVYTLPPSREEMTKNQVSLTCLVKGFYPSDIAVEWESNGQPENNYKTTPPVLDSDGSFFLYSKLTVDKSRWQQGNVFSCSVMHEALHNHYTQKSLSLSPGK

SEQ ID NO: 183 - protein, 356 aa, Artificial Sequence
  PR001780 HC
EVQLLESGGGLIQPGGSLRLSCAASGFTFSSFAMTWVRQAPGKGLEWVSTISGSGDNTYYADSVKGRFTISRDNSKNTLYLQMNSLRAEDTAVYFCAKEDTAVASDYYYNIDVWGQGTTVTVSSEPKSCDKTHTCPPCPAPELLGGPSVFLFPPKPKDTLMISRTPEVTCVVVDVSHEDPEVKFNWYVDGVEVHNAKTKPREEQYNSTYRVVSVLTVLHQDWLNGKEYKCKVSNKALPAPIEKTISKAKGQPREPQVYTLPPSREEMTKNQVSLTCLVKGFYPSDIAVEWESNGQPENNYKTTPPVLDSDGSFFLYSKLTVDKSRWQQGNVFSCSVMHEALHNHYTQKSLSLSPGK

SEQ ID NO: 184 - protein, 356 aa, Artificial Sequence
  PR001781 HC
EVQLLESGGGLVQLGGSLRLSCAASGFTFSSYAMTWVRQAPEKGLEWVSSISGSGGNTYYADSVKGRFTISRDNSKNTLYLQMNSLRAEDTAVYYCAKERTGTTGDYYYNVDVWGQGTTVTVSSEPKSCDKTHTCPPCPAPELLGGPSVFLFPPKPKDTLMISRTPEVTCVVVDVSHEDPEVKFNWYVDGVEVHNAKTKPREEQYNSTYRVVSVLTVLHQDWLNGKEYKCKVSNKALPAPIEKTISKAKGQPREPQVYTLPPSREEMTKNQVSLTCLVKGFYPSDIAVEWESNGQPENNYKTTPPVLDSDGSFFLYSKLTVDKSRWQQGNVFSCSVMHEALHNHYTQKSLSLSPGK

SEQ ID NO: 185 - protein, 356 aa, Artificial Sequence
  PR001830 HC
EVQLLESGGGLVQPGGSLRLSCTASGFTFSNYAMSWVRQAPEKGLEWVSSISGSGGSTFYADSVKGRFTISRDNSKNTLYLQMNSLRAEDTAVYFCAKEGSSETDDHYYNVDVWGQGTTVTVSSEPKSCDKTHTCPPCPAPELLGGPSVFLFPPKPKDTLMISRTPEVTCVVVDVSHEDPEVKFNWYVDGVEVHNAKTKPREEQYNSTYRVVSVLTVLHQDWLNGKEYKCKVSNKALPAPIEKTISKAKGQPREPQVYTLPPSREEMTKNQVSLTCLVKGFYPSDIAVEWESNGQPENNYKTTPPVLDSDGSFFLYSKLTVDKSRWQQGNVFSCSVMHEALHNHYTQKSLSLSPGK

SEQ ID NO: 186 - protein, 356 aa, Artificial Sequence
  PR001833 HC
EVQLLESGGGLVQPGGSLRLSCAASGFTFSSYAMSWVRQAPEKGLEWVSSISGSGGSTFYADSVKGRFTISRDNSKNTLYLQMNSLRAEDTAVYFCAKEGATETDDYHFNTDVWGQGTTVTVSSEPKSCDKTHTCPPCPAPELLGGPSVFLFPPKPKDTLMISRTPEVTCVVVDVSHEDPEVKFNWYVDGVEVHNAKTKPREEQYNSTYRVVSVLTVLHQDWLNGKEYKCKVSNKALPAPIEKTISKAKGQPREPQVYTLPPSREEMTKNQVSLTCLVKGFYPSDIAVEWESNGQPENNYKTTPPVLDSDGSFFLYSKLTVDKSRWQQGNVFSCSVMHEALHNHYTQKSLSLSPGK

SEQ ID NO: 187 - protein, 356 aa, Artificial Sequence
  PR001836 HC
EVQLLESGGGLVQPGGSLRLSCAASGFIFSNFAMTWVRQPPEKGLKWVSSINGSGFNTYYTDSVKGRFTISRDNSRNTLYLQMNRLTAEDTAVYFCAKEGSSETDDHYYNVDVWGQGTTVTVSSEPKSCDKTHTCPPCPAPELLGGPSVFLFPPKPKDTLMISRTPEVTCVVVDVSHEDPEVKFNWYVDGVEVHNAKTKPREEQYNSTYRVVSVLTVLHQDWLNGKEYKCKVSNKALPAPIEKTISKAKGQPREPQVYTLPPSREEMTKNQVSLTCLVKGFYPSDIAVEWESNGQPENNYKTTPPVLDSDGSFFLYSKLTVDKSRWQQGNVFSCSVMHEALHNHYTQKSLSLSPGK

SEQ ID NO: 188 - protein, 356 aa, Artificial Sequence
  PR001838 HC
EVQLLESGGGLVQPGGSLRLSCAASGFTFSNYAMSWFRQPPETGLKWVSSIDGSGGDTYYADSVKGRFTISRDNSKNTLYLQMNSLRAEDTAVYYCAKEGSHGTDDSHYDVDVWGQGTTVTVSSEPKSCDKTHTCPPCPAPELLGGPSVFLFPPKPKDTLMISRTPEVTCVVVDVSHEDPEVKFNWYVDGVEVHNAKTKPREEQYNSTYRVVSVLTVLHQDWLNGKEYKCKVSNKALPAPIEKTISKAKGQPREPQVYTLPPSREEMTKNQVSLTCLVKGFYPSDIAVEWESNGQPENNYKTTPPVLDSDGSFFLYSKLTVDKSRWQQGNVFSCSVMHEALHNHYTQKSLSLSPGK

SEQ ID NO: 189 - protein, 355 aa, Artificial Sequence
  PR001840 HC
EVQLVESGGGLVQPGGSLRLSCAASGFTFSSYWMHWVRQAPGKGLVWVSRINSDGSSTSYADSVQGRFTISRDNAKNTLYLQMNSLRAEDTAVYYCVRKGSSSYYHYSIEDDWGQGTLVTVSSEPKSCDKTHTCPPCPAPELLGGPSVFLFPPKPKDTLMISRTPEVTCVVVDVSHEDPEVKFNWYVDGVEVHNAKTKPREEQYNSTYRVVSVLTVLHQDWLNGKEYKCKVSNKALPAPIEKTISKAKGQPREPQVYTLPPSREEMTKNQVSLTCLVKGFYPSDIAVEWESNGQPENNYKTTPPVLDSDGSFFLYSKLTVDKSRWQQGNVFSCSVMHEALHNHYTQKSLSLSPGK

SEQ ID NO: 190 - protein, 356 aa, Artificial Sequence
  PR001842 HC
EVQLLESGGGLVQPGGSLRLSCAASGFTFSSYAMSWGRQAPGKGLEWVSAISGSGGSTYYADSVKGRFTISRDNSKNTLYLHMNSLRAEDTAVYYCAKEKVATTGDYYYDMDVWGQGTTVTVSSEPKSCDKTHTCPPCPAPELLGGPSVFLFPPKPKDTLMISRTPEVTCVVVDVSHEDPEVKFNWYVDGVEVHNAKTKPREEQYNSTYRVVSVLTVLHQDWLNGKEYKCKVSNKALPAPIEKTISKAKGQPREPQVYTLPPSREEMTKNQVSLTCLVKGFYPSDIAVEWESNGQPENNYKTTPPVLDSDGSFFLYSKLTVDKSRWQQGNVFSCSVMHEALHNHYTQKSLSLSPGK

SEQ ID NO: 191 - protein, 446 aa, Artificial Sequence
  PR002037 HC, PR002410 HC
QVQLVQSGAEVKKPGSSMRVSCKASEDTFSSYAISWVRQAPGQGLEWMGGTAPIFGTTNYAQKFQGRVTITADKSTSTAYMELSSLRSEDTAVYYCARGGPYFDYWGQGTLVTVSSASTKGPSVFPLAPSSKSTSGGTAALGCLVKDYFPEPVTVSWNSGALTSGVHTFPAVLQSSGLYSLSSVVTVPSSSLGTQTYICNVNHKPSNTKVDKKVEPKSCDKTHTCPPCPAPELLGGPSVFLFPPKPKDTLMISRTPEVTCVVVDVSHEDPEVKFNWYVDGVEVHNAKTKPREEQYNSTYRVVSVLTVLHQDWLNGKEYKCKVSNKALPAPIEKTISKAKGQPREPQVYTLPPSREEMTKNQVSLTCLVKGFYPSDIAVEWESNGQPENNYKTTPPVLDSDGSFFLYSKLTVDKSRWQQGNVFSCSVMHEALHNHYTQKSLSLSPGK

SEQ ID NO: 192 - protein, 449 aa, Artificial Sequence
  PR002408 HC
QVQLVESGGGVVQPGRSLRLSCAASGFTFRSFGMHWVRQAPGKGLEWVAVISYDASNEYYADSVKGRFIISRDNSKDTLYLQMNSLRAGDTAVYYCAKGGGLRWYFAYWGQGTLVTVSSASTKGPSVFPLAPSSKSTSGGTAALGCLVKDYFPEPVTVSWNSGALTSGVHTFPAVLQSSGLYSLSSVVTVPSSSLGTQTYICNVNHKPSNTKVDKKVEPKSCDKTHTCPPCPAPELLGGPSVFLFPPKPKDTLMISRTPEVTCVVVDVSHEDPEVKFNWYVDGVEVHNAKTKPREEQYNSTYRVVSVLTVLHQDWLNGKEYKCKVSNKALPAPIEKTISKAKGQPREPQVYTLPPSREEMTKNQVSLTCLVKGFYPSDIAVEWESNGQPENNYKTTPPVLDSDGSFFLYSKLTVDKSRWQQGNVFSCSVMHEALHNHYTQKSLSLSPGK

SEQ ID NO: 193 - protein, 356 aa, Artificial Sequence
  PR004469 HC
EVQLLESGGGLVQPGGSLRLSCAASGFTFSNYAMSWFRQPPETGLKWVSSIDASGGDTYYADSVKGRFTISRDNSKNTLYLQMNSLRAEDTAVYYCAKEGSHGTDDSHYDVDVWGQGTTVTVSSEPKSCDKTHTCPPCPAPELLGGPSVFLFPPKPKDTLMISRTPEVTCVVVDVSHEDPEVKFNWYVDGVEVHNAKTKPREEQYNSTYRVVSVLTVLHQDWLNGKEYKCKVSNKALPAPIEKTISKAKGQPREPQVYTLPPSREEMTKNQVSLTCLVKGFYPSDIAVEWESNGQPENNYKTTPPVLDSDGSFFLYSKLTVDKSRWQQGNVFSCSVMHEALHNHYTQKSLSLSPGK

SEQ ID NO: 194 - protein, 214 aa, Artificial Sequence
  PR000157 LC
DIQMTQSPSSLSASVGDRVTITCKASQGFNKYVAWYQQKPGKAPKLLIYYTSTLQPGVPSRFSGSGSGRDYTLTISSLQPEDFATYYCLQYGDLLYAFGQGTKVEIKRTVAAPSVFIFPPSDEQLKSGTASVVCLLNNFYPREAKVQWKVDNALQSGNSQESVTEQDSKDSTYSLSSTLTLSKADYEKHKVYACEVTHQGLSSPVTKSFNRGEC

SEQ ID NO: 195 - protein, 214 aa, Artificial Sequence
  PR000448 LC
EIVMTQSPATLSVSPGERATLSCRASQSISSILAWYQQKPGQAPRLLIYGASTRATGIPARFSGSGSGTEFTLTISSLQSEDFAVYYCQQYYNWPLTFGGGTKVEIKRTVAAPSVFIFPPSDEQLKSGTASVVCLLNNFYPREAKVQWKVDNALQSGNSQESVTEQDSKDSTYSLSSTLTLSKADYEKHKVYACEVTHQGLSSPVTKSFNRGEC

SEQ ID NO: 196 - protein, 214 aa, Artificial Sequence
  PR000483 LC
SYELTQPPSVSVSPGQTASITCSGDNIGDQYAHWYQQKPGQSPVLVIYQDKNRPSGIPERFSGSNSGNTATLTISGTQAMDEADYYCATYTGFGSLAVFGGGTKLTVLGQPKAAPSVTLFPPSSEELQANKATLVCLISDFYPGAVTVAWKADSSPVKAGVETTTPSKQSNNKYAASSYLSLTPEQWKSHRSYSCQVTHEGSTVEKTVAPTECS

SEQ ID NO: 197 - protein, 216 aa, Artificial Sequence
  PR000628 LC
EIVLTQSPATLSLSPGERATLSCRASQSVSSYLAWYQQKPGQAPRLLIYDASNRATGIPARFSGSGSGTDFTLTISSLEPEDFAVYYCQQRSNWPPALTFGGGTKVEIKRTVAAPSVFIFPPSDEQLKSGTASVVCLLNNFYPREAKVQWKVDNALQSGNSQESVTEQDSKDSTYSLSSTLTLSKADYEKHKVYACEVTHQGLSSPVTKSFNRGEC

SEQ ID NO: 198 - protein, 215 aa, Artificial Sequence
  PR001476 LC, PR002789 Chain, PR002790 Chain, PR002791 Chain, PR002792
EIVMTQSPATLSVSPGERATLSCRASQSISSNLGWYQQKPGQAPRLLIYGASTRATGIPARFSGSGSGTEFTLTISSLQSEDFAVYYCQQYNSWPPLTFGGGTKVEIKRTVAAPSVFIFPPSDEQLKSGTASVVCLLNNFYPREAKVQWKVDNALQSGNSQESVTEQDSKDSTYSLSSTLTLSKADYEKHKVYACEVTHQGLSSPVTKSFNRGEC

SEQ ID NO: 199 - protein, 214 aa, Artificial Sequence
  PR002037 LC
EIVMTQSPASLSVSPGERATLSCRASQSVSSNLAWYQQKPGQAPRLLIYGASTRATGIPARVSGGGSGTEFTLTISSLQSEDFAVYCCQQYKNWPFTFGPGTKLEIKRTVAAPSVFIFPPSDEQLKSGTASVVCLLNNFYPREAKVQWKVDNALQSGNSQESVTEQDSKDSTYSLSSTLTLSKADYEKHKVYACEVTHQGLSSPVTKSFNRGEC

SEQ ID NO: 200 - protein, 215 aa, Artificial Sequence
  PR002408 LC, PR003334 Chain, PR003335 Chain, PR003336 Chain, PR003337
EIVMTQSPATLSVSPGERATLSCRASQSISSNLGWYQQKPGQAPRLLIYGASTRATGIPARFSGSGSGTEFTLTISSLQSEDFAVYYCQQYQSWPPLTFGGGTKVEIKRTVAAPSVFIFPPSDEQLKSGTASVVCLLNNFYPREAKVQWKVDNALQSGNSQESVTEQDSKDSTYSLSSTLTLSKADYEKHKVYACEVTHQGLSSPVTKSFNRGEC

SEQ ID NO: 201 - protein, 214 aa, Artificial Sequence
  PR002410 LC, PR002972 Chain, PR004158 Chain, PR004160 Chain, PR004161
EIVMTQSPASLSVSPGERATLSCRASQSVSSNLAWYQQKPGQAPRLLIYGASTRATGIPARVSGGGSGTEFTLTISSLQSEDFAVYYCQQYKNWPFTFGPGTKLEIKRTVAAPSVFIFPPSDEQLKSGTASVVCLLNNFYPREAKVQWKVDNALQSGNSQESVTEQDSKDSTYSLSSTLTLSKADYEKHKVYACEVTHQGLSSPVTKSFNRGEC

SEQ ID NO: 202 - protein, 702 aa, Artificial Sequence
  PR002789 Chain
QVQLVESGGGVVQPGRSLRLSCAASGFTFRSFGMHWVRQAPGKGLEWVAVISYDGSNEYYADSVKGRFIISRDNSKDTLYLQMNSLRAGDTAVYYCAKGGGLRWYFAYWGQGTLVTVSSASTKGPSVFPLAPSSKSTSGGTAALGCLVKDYFPEPVTVSWNSGALTSGVHTFPAVLQSSGLYSLSSVVTVPSSSLGTQTYICNVNHKPSNTKVDKKVEPKSCDKTHTCPPCPAPEAAGGPSVFLFPPKPKDTLMISRTPEVTCVVVDVSHEDPEVKFNWYVDGVEVHNAKTKPREEQYNSTYRVVSVLTVLHQDWLNGKEYKCKVSNKALGAPIEKTISKAKGQPREPQVYTLPPSREEMTKNQVSLTCLVKGFYPSDIAVEWESNGQPENNYKTTPPVLDSDGSFFLYSKLTVDKSRWQQGNVFSCSVMHEALHNHYTQKSLSLSPGEPKSSDKTHTPPPPPRTQVQLQQWGAGLLKPSETLSLTCAVYGGSFSGYYWSWIRQPPGKGLEWIGEIQHSGSTDSNPSLKGRVTFSVDTSKNQFSLKLNSVTAADTAVYYCARLTGPFDYWGQGTLVTVSSGGGGSGGGGSGGGGSEIVMTQSPATLSVSPGERATLSCRASQSISSILAWYQQKPGQAPRLLIYGASTRATGIPARFSGSGSGTEFTLTISSLQSEDFAVYYCQQYYNWPLTFGGGTKVEIK

SEQ ID NO: 203 - protein, 589 aa, Artificial Sequence
  PR002790 Chain
QVQLVESGGGVVQPGRSLRLSCAASGFTFRSFGMHWVRQAPGKGLEWVAVISYDGSNEYYADSVKGRFIISRDNSKDTLYLQMNSLRAGDTAVYYCAKGGGLRWYFAYWGQGTLVTVSSASTKGPSVFPLAPSSKSTSGGTAALGCLVKDYFPEPVTVSWNSGALTSGVHTFPAVLQSSGLYSLSSVVTVPSSSLGTQTYICNVNHKPSNTKVDKKVEPKSCDKTHTCPPCPAPEAAGGPSVFLFPPKPKDTLMISRTPEVTCVVVDVSHEDPEVKFNWYVDGVEVHNAKTKPREEQYNSTYRVVSVLTVLHQDWLNGKEYKCKVSNKALGAPIEKTISKAKGQPREPQVYTLPPSREEMTKNQVSLTCLVKGFYPSDIAVEWESNGQPENNYKTTPPVLDSDGSFFLYSKLTVDKSRWQQGNVFSCSVMHEALHNHYTQKSLSLSPGEPKSSDKTHTPPPPPRTEVQLLESGGGLVQLGGSLRLSCAASGFTFSRYAMTWVRQAPEKGLEWVSSISGSGDDTYYGDSVKGRFTISRDNSQNTVYLQMNSLRAEDTAVYFCAKEKAGTTGDYYYNVDVWGQGTTVTVSS

SEQ ID NO: 204 - protein, 589 aa, Artificial Sequence
  PR002791 Chain
QVQLVESGGGVVQPGRSLRLSCAASGFTFRSFGMHWVRQAPGKGLEWVAVISYDGSNEYYADSVKGRFIISRDNSKDTLYLQMNSLRAGDTAVYYCAKGGGLRWYFAYWGQGTLVTVSSASTKGPSVFPLAPSSKSTSGGTAALGCLVKDYFPEPVTVSWNSGALTSGVHTFPAVLQSSGLYSLSSVVTVPSSSLGTQTYICNVNHKPSNTKVDKKVEPKSCDKTHTCPPCPAPEAAGGPSVFLFPPKPKDTLMISRTPEVTCVVVDVSHEDPEVKFNWYVDGVEVHNAKTKPREEQYNSTYRVVSVLTVLHQDWLNGKEYKCKVSNKALGAPIEKTISKAKGQPREPQVYTLPPSREEMTKNQVSLTCLVKGFYPSDIAVEWESNGQPENNYKTTPPVLDSDGSFFLYSKLTVDKSRWQQGNVFSCSVMHEALHNHYTQKSLSLSPGEPKSSDKTHTPPPPPRTEVQLVESGGGVVQPGGSLRLSCAASGFTFSNYAMTWVRQAPEKGLEWVSSISGSGVSTYYADSVKGRFTISRDNSKNTLYLQMTRLTAEDTAVYFCAKEGSSETDDHYYNVDVWGQGTTVTVSS

SEQ ID NO: 205 - protein, 589 aa, Artificial Sequence
  PR002792 Chain
QVQLVESGGGVVQPGRSLRLSCAASGFTFRSFGMHWVRQAPGKGLEWVAVISYDGSNEYYADSVKGRFIISRDNSKDTLYLQMNSLRAGDTAVYYCAKGGGLRWYFAYWGQGTLVTVSSASTKGPSVFPLAPSSKSTSGGTAALGCLVKDYFPEPVTVSWNSGALTSGVHTFPAVLQSSGLYSLSSVVTVPSSSLGTQTYICNVNHKPSNTKVDKKVEPKSCDKTHTCPPCPAPEAAGGPSVFLFPPKPKDTLMISRTPEVTCVVVDVSHEDPEVKFNWYVDGVEVHNAKTKPREEQYNSTYRVVSVLTVLHQDWLNGKEYKCKVSNKALGAPIEKTISKAKGQPREPQVYTLPPSREEMTKNQVSLTCLVKGFYPSDIAVEWESNGQPENNYKTTPPVLDSDGSFFLYSKLTVDKSRWQQGNVFSCSVMHEALHNHYTQKSLSLSPGEPKSSDKTHTPPPPPRTEVQLLESGGGLVQPGGSLRLSCTASGFTFSNYAMSWVRQAPEKGLEWVSSISGSGGSTFYADSVKGRFTISRDNSKNTLYLQMNRLTAEDTAVYYCAKEGSNGTDDYHYDIDVWGQGTTVTVSS

SEQ ID NO: 206 - protein, 589 aa, Artificial Sequence
  PR002793 Chain
QVQLVESGGGVVQPGRSLRLSCAASGFTFRSFGMHWVRQAPGKGLEWVAVISYDGSNEYYADSVKGRFIISRDNSKDTLYLQMNSLRAGDTAVYYCAKGGGLRWYFAYWGQGTLVTVSSASTKGPSVFPLAPSSKSTSGGTAALGCLVKDYFPEPVTVSWNSGALTSGVHTFPAVLQSSGLYSLSSVVTVPSSSLGTQTYICNVNHKPSNTKVDKKVEPKSCDKTHTCPPCPAPEAAGGPSVFLFPPKPKDTLMISRTPEVTCVVVDVSHEDPEVKFNWYVDGVEVHNAKTKPREEQYNSTYRVVSVLTVLHQDWLNGKEYKCKVSNKALGAPIEKTISKAKGQPREPQVYTLPPSREEMTKNQVSLTCLVKGFYPSDIAVEWESNGQPENNYKTTPPVLDSDGSFFLYSKLTVDKSRWQQGNVFSCSVMHEALHNHYTQKSLSLSPGEPKSSDKTHTPPPPPRTEVQLLESGGGLVQPGGSLRLSCAASGFTFSSYAMSWVRQAPEKGLEWVSAISGGGGSTYYADSVKGRFTISRDNSKNTLYLQMDSLKAEDTAVYYCAKEGTTETDDYHYNMDVWGQGTTVTVSS

SEQ ID NO: 207 - protein, 591 aa, Artificial Sequence
  PR002794 Chain
QVQLVESGGGVVQPGRSLRLSCAASGFTFRSFGMHWVRQAPGKGLEWVAVISYDGSNEYYADSVKGRFIISRDNSKDTLYLQMNSLRAGDTAVYYCAKGGGLRWYFAYWGQGTLVTVSSASTKGPSVFPLAPSSKSTSGGTAALGCLVKDYFPEPVTVSWNSGALTSGVHTFPAVLQSSGLYSLSSVVTVPSSSLGTQTYICNVNHKPSNTKVDKKVEPKSCDKTHTCPPCPAPEAAGGPSVFLFPPKPKDTLMISRTPEVTCVVVDVSHEDPEVKFNWYVDGVEVHNAKTKPREEQYNSTYRVVSVLTVLHQDWLNGKEYKCKVSNKALGAPIEKTISKAKGQPREPQVYTLPPSREEMTKNQVSLTCLVKGFYPSDIAVEWESNGQPENNYKTTPPVLDSDGSFFLYSKLTVDKSRWQQGNVFSCSVMHEALHNHYTQKSLSLSPGEPKSSDKTHTPPPPPRTEVQLVETGGGLIQPGGSLRLSCAASGFTVSSNYMSWVRQAPGKGLEWVSVIYSDGSTYYADSVKGRFTISRDNSKNTLYLQMNSLRAEDTAVYYCARDRYYGSGNYPTAYYGMDVRGQGTTVTVSS

SEQ ID NO: 208 - protein, 589 aa, Artificial Sequence
  PR002795 Chain
QVQLVESGGGVVQPGRSLRLSCAASGFTFRSFGMHWVRQAPGKGLEWVAVISYDGSNEYYADSVKGRFIISRDNSKDTLYLQMNSLRAGDTAVYYCAKGGGLRWYFAYWGQGTLVTVSSASTKGPSVFPLAPSSKSTSGGTAALGCLVKDYFPEPVTVSWNSGALTSGVHTFPAVLQSSGLYSLSSVVTVPSSSLGTQTYICNVNHKPSNTKVDKKVEPKSCDKTHTCPPCPAPEAAGGPSVFLFPPKPKDTLMISRTPEVTCVVVDVSHEDPEVKFNWYVDGVEVHNAKTKPREEQYNSTYRVVSVLTVLHQDWLNGKEYKCKVSNKALGAPIEKTISKAKGQPREPQVYTLPPSREEMTKNQVSLTCLVKGFYPSDIAVEWESNGQPENNYKTTPPVLDSDGSFFLYSKLTVDKSRWQQGNVFSCSVMHEALHNHYTQKSLSLSPGEPKSSDKTHTPPPPPRTEVQLLESGGGLVQPGGSLRLSCAASGFTFSNYAMTWVRQAPGKGLEWVSSISGSGDSTYYADSVKGRFTISRDNSKNTLYLQMNSLRAEDTAVYYCAKEGTGTTSDYYYNVDVWGQGTTVTVSS

SEQ ID NO: 209 - protein, 589 aa, Artificial Sequence
  PR002798 Chain
QVQLVESGGGVVQPGRSLRLSCAASGFTFRSFGMHWVRQAPGKGLEWVAVISYDGSNEYYADSVKGRFIISRDNSKDTLYLQMNSLRAGDTAVYYCAKGGGLRWYFAYWGQGTLVTVSSASTKGPSVFPLAPSSKSTSGGTAALGCLVKDYFPEPVTVSWNSGALTSGVHTFPAVLQSSGLYSLSSVVTVPSSSLGTQTYICNVNHKPSNTKVDKKVEPKSCDKTHTCPPCPAPEAAGGPSVFLFPPKPKDTLMISRTPEVTCVVVDVSHEDPEVKFNWYVDGVEVHNAKTKPREEQYNSTYRVVSVLTVLHQDWLNGKEYKCKVSNKALGAPIEKTISKAKGQPREPQVYTLPPSREEMTKNQVSLTCLVKGFYPSDIAVEWESNGQPENNYKTTPPVLDSDGSFFLYSKLTVDKSRWQQGNVFSCSVMHEALHNHYTQKSLSLSPGEPKSSDKTHTPPPPPRTEVQLVESGGGLVQPGGSLRLSCAASGFTFSSFAMTWVRQAPEKGLEWVSTISGSGDTTYYADSVKGRFTISRDSSKNTLYLQMNSLRAEDSAVYFCAKEATAMASDYYYGVDVWGQGTTVTVSS

SEQ ID NO: 210 - protein, 589 aa, Artificial Sequence
  PR002800 Chain
QVQLVESGGGVVQPGRSLRLSCAASGFTFRSFGMHWVRQAPGKGLEWVAVISYDGSNEYYADSVKGRFIISRDNSKDTLYLQMNSLRAGDTAVYYCAKGGGLRWYFAYWGQGTLVTVSSASTKGPSVFPLAPSSKSTSGGTAALGCLVKDYFPEPVTVSWNSGALTSGVHTFPAVLQSSGLYSLSSVVTVPSSSLGTQTYICNVNHKPSNTKVDKKVEPKSCDKTHTCPPCPAPEAAGGPSVFLFPPKPKDTLMISRTPEVTCVVVDVSHEDPEVKFNWYVDGVEVHNAKTKPREEQYNSTYRVVSVLTVLHQDWLNGKEYKCKVSNKALGAPIEKTISKAKGQPREPQVYTLPPSREEMTKNQVSLTCLVKGFYPSDIAVEWESNGQPENNYKTTPPVLDSDGSFFLYSKLTVDKSRWQQGNVFSCSVMHEALHNHYTQKSLSLSPGEPKSSDKTHTPPPPPRTEVQLLESGGGLIQPGGSLRLSCAASGFTFSSFAMTWVRQAPGKGLEWVSTISGSGDNTYYADSVKGRFTISRDNSKNTLYLQMNSLRAEDTAVYFCAKEDTAVASDYYYNIDVWGQGTTVTVSS

SEQ ID NO: 211 - protein, 589 aa, Artificial Sequence
  PR002801 Chain
QVQLVESGGGVVQPGRSLRLSCAASGFTFRSFGMHWVRQAPGKGLEWVAVISYDGSNEYYADSVKGRFIISRDNSKDTLYLQMNSLRAGDTAVYYCAKGGGLRWYFAYWGQGTLVTVSSASTKGPSVFPLAPSSKSTSGGTAALGCLVKDYFPEPVTVSWNSGALTSGVHTFPAVLQSSGLYSLSSVVTVPSSSLGTQTYICNVNHKPSNTKVDKKVEPKSCDKTHTCPPCPAPEAAGGPSVFLFPPKPKDTLMISRTPEVTCVVVDVSHEDPEVKFNWYVDGVEVHNAKTKPREEQYNSTYRVVSVLTVLHQDWLNGKEYKCKVSNKALGAPIEKTISKAKGQPREPQVYTLPPSREEMTKNQVSLTCLVKGFYPSDIAVEWESNGQPENNYKTTPPVLDSDGSFFLYSKLTVDKSRWQQGNVFSCSVMHEALHNHYTQKSLSLSPGEPKSSDKTHTPPPPPRTEVQLLESGGGLVQLGGSLRLSCAASGFTFSSYAMTWVRQAPEKGLEWVSSISGSGGNTYYADSVKGRFTISRDNSKNTLYLQMNSLRAEDTAVYYCAKERTGTTGDYYYNVDVWGQGTTVTVSS

SEQ ID NO: 212 - protein, 589 aa, Artificial Sequence
  PR002802 Chain
QVQLVESGGGVVQPGRSLRLSCAASGFTFRSFGMHWVRQAPGKGLEWVAVISYDGSNEYYADSVKGRFIISRDNSKDTLYLQMNSLRAGDTAVYYCAKGGGLRWYFAYWGQGTLVTVSSASTKGPSVFPLAPSSKSTSGGTAALGCLVKDYFPEPVTVSWNSGALTSGVHTFPAVLQSSGLYSLSSVVTVPSSSLGTQTYICNVNHKPSNTKVDKKVEPKSCDKTHTCPPCPAPEAAGGPSVFLFPPKPKDTLMISRTPEVTCVVVDVSHEDPEVKFNWYVDGVEVHNAKTKPREEQYNSTYRVVSVLTVLHQDWLNGKEYKCKVSNKALGAPIEKTISKAKGQPREPQVYTLPPSREEMTKNQVSLTCLVKGFYPSDIAVEWESNGQPENNYKTTPPVLDSDGSFFLYSKLTVDKSRWQQGNVFSCSVMHEALHNHYTQKSLSLSPGEPKSSDKTHTPPPPPRTEVQLLESGGGLVQPGGSLRLSCTASGFTFSNYAMSWVRQAPEKGLEWVSSISGSGGSTFYADSVKGRFTISRDNSKNTLYLQMNSLRAEDTAVYFCAKEGSSETDDHYYNVDVWGQGTTVTVSS

SEQ ID NO: 213 - protein, 589 aa, Artificial Sequence
  PR002804 Chain
QVQLVESGGGVVQPGRSLRLSCAASGFTFRSFGMHWVRQAPGKGLEWVAVISYDGSNEYYADSVKGRFIISRDNSKDTLYLQMNSLRAGDTAVYYCAKGGGLRWYFAYWGQGTLVTVSSASTKGPSVFPLAPSSKSTSGGTAALGCLVKDYFPEPVTVSWNSGALTSGVHTFPAVLQSSGLYSLSSVVTVPSSSLGTQTYICNVNHKPSNTKVDKKVEPKSCDKTHTCPPCPAPEAAGGPSVFLFPPKPKDTLMISRTPEVTCVVVDVSHEDPEVKFNWYVDGVEVHNAKTKPREEQYNSTYRVVSVLTVLHQDWLNGKEYKCKVSNKALGAPIEKTISKAKGQPREPQVYTLPPSREEMTKNQVSLTCLVKGFYPSDIAVEWESNGQPENNYKTTPPVLDSDGSFFLYSKLTVDKSRWQQGNVFSCSVMHEALHNHYTQKSLSLSPGEPKSSDKTHTPPPPPRTEVQLLESGGGLVQPGGSLRLSCAASGFTFSSYAMSWVRQAPEKGLEWVSSISGSGGSTFYADSVKGRFTISRDNSKNTLYLQMNSLRAEDTAVYFCAKEGATETDDYHFNTDVWGQGTTVTVSS

SEQ ID NO: 214 - protein, 589 aa, Artificial Sequence
  PR002805 Chain
QVQLVESGGGVVQPGRSLRLSCAASGFTFRSFGMHWVRQAPGKGLEWVAVISYDGSNEYYADSVKGRFIISRDNSKDTLYLQMNSLRAGDTAVYYCAKGGGLRWYFAYWGQGTLVTVSSASTKGPSVFPLAPSSKSTSGGTAALGCLVKDYFPEPVTVSWNSGALTSGVHTFPAVLQSSGLYSLSSVVTVPSSSLGTQTYICNVNHKPSNTKVDKKVEPKSCDKTHTCPPCPAPEAAGGPSVFLFPPKPKDTLMISRTPEVTCVVVDVSHEDPEVKFNWYVDGVEVHNAKTKPREEQYNSTYRVVSVLTVLHQDWLNGKEYKCKVSNKALGAPIEKTISKAKGQPREPQVYTLPPSREEMTKNQVSLTCLVKGFYPSDIAVEWESNGQPENNYKTTPPVLDSDGSFFLYSKLTVDKSRWQQGNVFSCSVMHEALHNHYTQKSLSLSPGEPKSSDKTHTPPPPPRTEVQLLESGGGLVQPGGSLRLSCAASGFIFSNFAMTWVRQPPEKGLKWVSSINGSGFNTYYTDSVKGRFTISRDNSRNTLYLQMNRLTAEDTAVYFCAKEGSSETDDHYYNVDVWGQGTTVTVSS

SEQ ID NO: 215 - protein, 589 aa, Artificial Sequence
  PR002806 Chain
QVQLVESGGGVVQPGRSLRLSCAASGFTFRSFGMHWVRQAPGKGLEWVAVISYDGSNEYYADSVKGRFIISRDNSKDTLYLQMNSLRAGDTAVYYCAKGGGLRWYFAYWGQGTLVTVSSASTKGPSVFPLAPSSKSTSGGTAALGCLVKDYFPEPVTVSWNSGALTSGVHTFPAVLQSSGLYSLSSVVTVPSSSLGTQTYICNVNHKPSNTKVDKKVEPKSCDKTHTCPPCPAPEAAGGPSVFLFPPKPKDTLMISRTPEVTCVVVDVSHEDPEVKFNWYVDGVEVHNAKTKPREEQYNSTYRVVSVLTVLHQDWLNGKEYKCKVSNKALGAPIEKTISKAKGQPREPQVYTLPPSREEMTKNQVSLTCLVKGFYPSDIAVEWESNGQPENNYKTTPPVLDSDGSFFLYSKLTVDKSRWQQGNVFSCSVMHEALHNHYTQKSLSLSPGEPKSSDKTHTPPPPPRTEVQLLESGGGLVQPGGSLRLSCAASGFTFSNYAMSWFRQPPETGLKWVSSIDGSGGDTYYADSVKGRFTISRDNSKNTLYLQMNSLRAEDTAVYYCAKEGSHGTDDSHYDVDVWGQGTTVTVSS

SEQ ID NO: 216 - protein, 589 aa, Artificial Sequence
  PR002808 Chain
QVQLVESGGGVVQPGRSLRLSCAASGFTFRSFGMHWVRQAPGKGLEWVAVISYDGSNEYYADSVKGRFIISRDNSKDTLYLQMNSLRAGDTAVYYCAKGGGLRWYFAYWGQGTLVTVSSASTKGPSVFPLAPSSKSTSGGTAALGCLVKDYFPEPVTVSWNSGALTSGVHTFPAVLQSSGLYSLSSVVTVPSSSLGTQTYICNVNHKPSNTKVDKKVEPKSCDKTHTCPPCPAPEAAGGPSVFLFPPKPKDTLMISRTPEVTCVVVDVSHEDPEVKFNWYVDGVEVHNAKTKPREEQYNSTYRVVSVLTVLHQDWLNGKEYKCKVSNKALGAPIEKTISKAKGQPREPQVYTLPPSREEMTKNQVSLTCLVKGFYPSDIAVEWESNGQPENNYKTTPPVLDSDGSFFLYSKLTVDKSRWQQGNVFSCSVMHEALHNHYTQKSLSLSPGEPKSSDKTHTPPPPPRTEVQLLESGGGLVQPGGSLRLSCAASGFTFSSYAMSWGRQAPGKGLEWVSAISGSGGSTYYADSVKGRFTISRDNSKNTLYLHMNSLRAEDTAVYYCAKEKVATTGDYYYDMDVWGQGTTVTVSS

SEQ ID NO: 217 - protein, 699 aa, Artificial Sequence
  PR002972 Chain
QVQLVQSGAEVKKPGSSMRVSCKASEDTFSSYAISWVRQAPGQGLEWMGGTAPIFGTTNYAQKFQGRVTITADKSTSTAYMELSSLRSEDTAVYYCARGGPYFDYWGQGTLVTVSSASTKGPSVFPLAPSSKSTSGGTAALGCLVKDYFPEPVTVSWNSGALTSGVHTFPAVLQSSGLYSLSSVVTVPSSSLGTQTYICNVNHKPSNTKVDKKVEPKSCDKTHTCPPCPAPEAAGGPSVFLFPPKPKDTLMISRTPEVTCVVVDVSHEDPEVKFNWYVDGVEVHNAKTKPREEQYNSTYRVVSVLTVLHQDWLNGKEYKCKVSNKALGAPIEKTISKAKGQPREPQVYTLPPSREEMTKNQVSLTCLVKGFYPSDIAVEWESNGQPENNYKTTPPVLDSDGSFFLYSKLTVDKSRWQQGNVFSCSVMHEALHNHYTQKSLSLSPGEPKSSDKTHTPPPPPRTQVQLQQWGAGLLKPSETLSLTCAVYGGSFSGYYWSWIRQPPGKGLEWIGEIQHSGSTDSNPSLKGRVTFSVDTSKNQFSLKLNSVTAADTAVYYCARLTGPFDYWGQGTLVTVSSGGGGSGGGGSGGGGSEIVMTQSPATLSVSPGERATLSCRASQSISSILAWYQQKPGQAPRLLIYGASTRATGIPARFSGSGSGTEFTLTISSLQSEDFAVYYCQQYYNWPLTFGGGTKVEIK

SEQ ID NO: 218 - protein, 589 aa, Artificial Sequence
  PR003334 Chain
QVQLVESGGGVVQPGRSLRLSCAASGFTFRSFGMHWVRQAPGKGLEWVAVISYDASNEYYADSVKGRFIISRDNSKDTLYLQMNSLRAGDTAVYYCAKGGGLRWYFAYWGQGTLVTVSSASTKGPSVFPLAPSSKSTSGGTAALGCLVKDYFPEPVTVSWNSGALTSGVHTFPAVLQSSGLYSLSSVVTVPSSSLGTQTYICNVNHKPSNTKVDKKVEPKSCDKTHTCPPCPAPEAAGGPSVFLFPPKPKDTLMISRTPEVTCVVVDVSHEDPEVKFNWYVDGVEVHNAKTKPREEQYNSTYRVVSVLTVLHQDWLNGKEYKCKVSNKALPAPIEKTISKAKGQPREPQVYTLPPSREEMTKNQVSLTCLVKGFYPSDIAVEWESNGQPENNYKTTPPVLDSDGSFFLYSKLTVDKSRWQQGNVFSCSVMHEALHNHYTQKSLSLSPGEPKSSDKTHTPPPPPRTEVQLLESGGGLVQLGGSLRLSCAASGFTFSRYAMTWVRQAPEKGLEWVSSISGSGDDTYYGDSVKGRFTISRDNSQNTVYLQMNSLRAEDTAVYFCAKEKAGTTGDYYYNVDVWGQGTTVTVSS

SEQ ID NO: 219 - protein, 589 aa, Artificial Sequence
  PR003335 Chain
QVQLVESGGGVVQPGRSLRLSCAASGFTFRSFGMHWVRQAPGKGLEWVAVISYDASNEYYADSVKGRFIISRDNSKDTLYLQMNSLRAGDTAVYYCAKGGGLRWYFAYWGQGTLVTVSSASTKGPSVFPLAPSSKSTSGGTAALGCLVKDYFPEPVTVSWNSGALTSGVHTFPAVLQSSGLYSLSSVVTVPSSSLGTQTYICNVNHKPSNTKVDKKVEPKSCDKTHTCPPCPAPEAAGGPSVFLFPPKPKDTLMISRTPEVTCVVVDVSHEDPEVKFNWYVDGVEVHNAKTKPREEQYNSTYRVVSVLTVLHQDWLNGKEYKCKVSNKALPAPIEKTISKAKGQPREPQVYTLPPSREEMTKNQVSLTCLVKGFYPSDIAVEWESNGQPENNYKTTPPVLDSDGSFFLYSKLTVDKSRWQQGNVFSCSVMHEALHNHYTQKSLSLSPGEPKSSDKTHTPPPPPRTEVQLVESGGGVVQPGGSLRLSCAASGFTFSNYAMTWVRQAPEKGLEWVSSISGSGVSTYYADSVKGRFTISRDNSKNTLYLQMTRLTAEDTAVYFCAKEGSSETDDHYYNVDVWGQGTTVTVSS

SEQ ID NO: 220 - protein, 589 aa, Artificial Sequence
  PR003336 Chain
QVQLVESGGGVVQPGRSLRLSCAASGFTFRSFGMHWVRQAPGKGLEWVAVISYDASNEYYADSVKGRFIISRDNSKDTLYLQMNSLRAGDTAVYYCAKGGGLRWYFAYWGQGTLVTVSSASTKGPSVFPLAPSSKSTSGGTAALGCLVKDYFPEPVTVSWNSGALTSGVHTFPAVLQSSGLYSLSSVVTVPSSSLGTQTYICNVNHKPSNTKVDKKVEPKSCDKTHTCPPCPAPEAAGGPSVFLFPPKPKDTLMISRTPEVTCVVVDVSHEDPEVKFNWYVDGVEVHNAKTKPREEQYNSTYRVVSVLTVLHQDWLNGKEYKCKVSNKALPAPIEKTISKAKGQPREPQVYTLPPSREEMTKNQVSLTCLVKGFYPSDIAVEWESNGQPENNYKTTPPVLDSDGSFFLYSKLTVDKSRWQQGNVFSCSVMHEALHNHYTQKSLSLSPGEPKSSDKTHTPPPPPRTEVQLLESGGGLVQPGGSLRLSCTASGFTFSNYAMSWVRQAPEKGLEWVSSISGSGGSTFYADSVKGRFTISRDNSKNTLYLQMNSLRAEDTAVYFCAKEGSSETDDHYYNVDVWGQGTTVTVSS

SEQ ID NO: 221 - protein, 589 aa, Artificial Sequence
  PR003337 Chain
QVQLVESGGGVVQPGRSLRLSCAASGFTFRSFGMHWVRQAPGKGLEWVAVISYDASNEYYADSVKGRFIISRDNSKDTLYLQMNSLRAGDTAVYYCAKGGGLRWYFAYWGQGTLVTVSSASTKGPSVFPLAPSSKSTSGGTAALGCLVKDYFPEPVTVSWNSGALTSGVHTFPAVLQSSGLYSLSSVVTVPSSSLGTQTYICNVNHKPSNTKVDKKVEPKSCDKTHTCPPCPAPEAAGGPSVFLFPPKPKDTLMISRTPEVTCVVVDVSHEDPEVKFNWYVDGVEVHNAKTKPREEQYNSTYRVVSVLTVLHQDWLNGKEYKCKVSNKALPAPIEKTISKAKGQPREPQVYTLPPSREEMTKNQVSLTCLVKGFYPSDIAVEWESNGQPENNYKTTPPVLDSDGSFFLYSKLTVDKSRWQQGNVFSCSVMHEALHNHYTQKSLSLSPGEPKSSDKTHTPPPPPRTEVQLLESGGGLVQPGGSLRLSCAASGFTFSSYAMSWVRQAPEKGLEWVSSISGSGGSTFYADSVKGRFTISRDNSKNTLYLQMNSLRAEDTAVYFCAKEGATETDDYHFNTDVWGQGTTVTVSS

SEQ ID NO: 222 - protein, 589 aa, Artificial Sequence
  PR003338 Chain
QVQLVESGGGVVQPGRSLRLSCAASGFTFRSFGMHWVRQAPGKGLEWVAVISYDASNEYYADSVKGRFIISRDNSKDTLYLQMNSLRAGDTAVYYCAKGGGLRWYFAYWGQGTLVTVSSASTKGPSVFPLAPSSKSTSGGTAALGCLVKDYFPEPVTVSWNSGALTSGVHTFPAVLQSSGLYSLSSVVTVPSSSLGTQTYICNVNHKPSNTKVDKKVEPKSCDKTHTCPPCPAPEAAGGPSVFLFPPKPKDTLMISRTPEVTCVVVDVSHEDPEVKFNWYVDGVEVHNAKTKPREEQYNSTYRVVSVLTVLHQDWLNGKEYKCKVSNKALPAPIEKTISKAKGQPREPQVYTLPPSREEMTKNQVSLTCLVKGFYPSDIAVEWESNGQPENNYKTTPPVLDSDGSFFLYSKLTVDKSRWQQGNVFSCSVMHEALHNHYTQKSLSLSPGEPKSSDKTHTPPPPPRTEVQLLESGGGLVQPGGSLRLSCAASGFTFSNYAMSWFRQPPETGLKWVSSIDASGGDTYYADSVKGRFTISRDNSKNTLYLQMNSLRAEDTAVYYCAKEGSHGTDDSHYDVDVWGQGTTVTVSS

SEQ ID NO: 223 - protein, 713 aa, Artificial Sequence
  PR003487 Chain
QVQLVESGGGVVQPGRSLRLSCAASGFTFRSFGMHWVRQAPGKGLEWVAVISYDASNEYYADSVKGRFIISRDNSKDTLYLQMNSLRAGDTAVYYCAKGGGLRWYFAYWGQGTLVTVSSASTKGPSVFPLAPSSKSTSGGTAALGCLVKDYFPEPVTVSWNSGALTSGVHTFPAVLQSSGLYSLSSVVTVPSSSLGTQTYICNVNHKPSNTKVDKKVEPKSCDKTHTCPPCPAPEAAGGPSVFLFPPKPKDTLMISRTPEVTCVVVDVSHEDPEVKFNWYVDGVEVHNAKTKPREEQYNSTYRVVSVLTVLHQDWLNGKEYKCKVSNKALPAPIEKTISKAKGQPREPQVYTLPPSREEMTKNQVSLTCLVKGFYPSDIAVEWESNGQPENNYKTTPPVLDSDGSFFLYSKLTVDKSRWQQGNVFSCSVMHEALHNHYTQKSLSLSPGEPKSSDKTHTPPPPPRTEVQLVESGGGVVQPGGSLRLSCAASGFTFSNYAMTWVRQAPEKGLEWVSSISGSGVSTYYADSVKGRFTISRDNSKNTLYLQMTRLTAEDTAVYFCAKEGSSETDDHYYNVDVWGQGTTVTVSSEVQLVESGGGVVQPGGSLRLSCAASGFTFSNYAMTWVRQAPEKGLEWVSSISGSGVSTYYADSVKGRFTISRDNSKNTLYLQMTRLTAEDTAVYFCAKEGSSETDDHYYNVDVWGQGTTVTVSS

SEQ ID NO: 224 - protein, 718 aa, Artificial Sequence
  PR003488 Chain
QVQLVESGGGVVQPGRSLRLSCAASGFTFRSFGMHWVRQAPGKGLEWVAVISYDASNEYYADSVKGRFIISRDNSKDTLYLQMNSLRAGDTAVYYCAKGGGLRWYFAYWGQGTLVTVSSASTKGPSVFPLAPSSKSTSGGTAALGCLVKDYFPEPVTVSWNSGALTSGVHTFPAVLQSSGLYSLSSVVTVPSSSLGTQTYICNVNHKPSNTKVDKKVEPKSCDKTHTCPPCPAPEAAGGPSVFLFPPKPKDTLMISRTPEVTCVVVDVSHEDPEVKFNWYVDGVEVHNAKTKPREEQYNSTYRVVSVLTVLHQDWLNGKEYKCKVSNKALPAPIEKTISKAKGQPREPQVYTLPPSREEMTKNQVSLTCLVKGFYPSDIAVEWESNGQPENNYKTTPPVLDSDGSFFLYSKLTVDKSRWQQGNVFSCSVMHEALHNHYTQKSLSLSPGEPKSSDKTHTPPPPPRTEVQLVESGGGVVQPGGSLRLSCAASGFTFSNYAMTWVRQAPEKGLEWVSSISGSGVSTYYADSVKGRFTISRDNSKNTLYLQMTRLTAEDTAVYFCAKEGSSETDDHYYNVDVWGQGTTVTVSSGGGGSEVQLVESGGGVVQPGGSLRLSCAASGFTFSNYAMTWVRQAPEKGLEWVSSISGSGVSTYYADSVKGRFTISRDNSKNTLYLQMTRLTAEDTAVYFCAKEGSSETDDHYYNVDVWGQGTTVTVSS

SEQ ID NO: 225 - protein, 728 aa, Artificial Sequence
  PR003489 Chain
QVQLVESGGGVVQPGRSLRLSCAASGFTFRSFGMHWVRQAPGKGLEWVAVISYDASNEYYADSVKGRFIISRDNSKDTLYLQMNSLRAGDTAVYYCAKGGGLRWYFAYWGQGTLVTVSSASTKGPSVFPLAPSSKSTSGGTAALGCLVKDYFPEPVTVSWNSGALTSGVHTFPAVLQSSGLYSLSSVVTVPSSSLGTQTYICNVNHKPSNTKVDKKVEPKSCDKTHTCPPCPAPEAAGGPSVFLFPPKPKDTLMISRTPEVTCVVVDVSHEDPEVKFNWYVDGVEVHNAKTKPREEQYNSTYRVVSVLTVLHQDWLNGKEYKCKVSNKALPAPIEKTISKAKGQPREPQVYTLPPSREEMTKNQVSLTCLVKGFYPSDIAVEWESNGQPENNYKTTPPVLDSDGSFFLYSKLTVDKSRWQQGNVFSCSVMHEALHNHYTQKSLSLSPGEPKSSDKTHTPPPPPRTEVQLVESGGGVVQPGGSLRLSCAASGFTFSNYAMTWVRQAPEKGLEWVSSISGSGVSTYYADSVKGRFTISRDNSKNTLYLQMTRLTAEDTAVYFCAKEGSSETDDHYYNVDVWGQGTTVTVSSGGGGSGGGGSGGGGSEVQLVESGGGVVQPGGSLRLSCAASGFTFSNYAMTWVRQAPEKGLEWVSSISGSGVSTYYADSVKGRFTISRDNSKNTLYLQMTRLTAEDTAVYFCAKEGSSETDDHYYNVDVWGQGTTVTVSS

SEQ ID NO: 226 - protein, 715 aa, Artificial Sequence
  PR004158 Chain
QVQLVQSGAEVKKPGSSMRVSCKASEDTFSSYAISWVRQAPGQGLEWMGGTAPIFGTTNYAQKFQGRVTITADKSTSTAYMELSSLRSEDTAVYYCARGGPYFDYWGQGTLVTVSSASTKGPSVFPLAPSSKSTSGGTAALGCLVKDYFPEPVTVSWNSGALTSGVHTFPAVLQSSGLYSLSSVVTVPSSSLGTQTYICNVNHKPSNTKVDKKVEPKSCDKTHTCPPCPAPEAAGGPSVFLFPPKPKDTLMISRTPEVTCVVVDVSHEDPEVKFNWYVDGVEVHNAKTKPREEQYNSTYRVVSVLTVLHQDWLNGKEYKCKVSNKALPAPIEKTISKAKGQPREPQVYTLPPSREEMTKNQVSLTCLVKGFYPSDIAVEWESNGQPENNYKTTPPVLDSDGSFFLYSKLTVDKSRWQQGNVFSCSVMHEALHNHYTQKSLSLSPGEPKSSDKTHTPPPPPRTEVQLVESGGGVVQPGGSLRLSCAASGFTFSNYAMTWVRQAPEKGLEWVSSISGSGVSTYYADSVKGRFTISRDNSKNTLYLQMTRLTAEDTAVYFCAKEGSSETDDHYYNVDVWGQGTTVTVSSGGGGSEVQLVESGGGVVQPGGSLRLSCAASGFTFSNYAMTWVRQAPEKGLEWVSSISGSGVSTYYADSVKGRFTISRDNSKNTLYLQMTRLTAEDTAVYFCAKEGSSETDDHYYNVDVWGQGTTVTVSS

SEQ ID NO: 227 - protein, 446 aa, Artificial Sequence
  PR004160 Chain, PR004161 Chain, PR004181 Chain, PR004182 Chain
QVQLVQSGAEVKKPGSSMRVSCKASEDTFSSYAISWVRQAPGQGLEWMGGTAPIFGTTNYAQKFQGRVTITADKSTSTAYMELSSLRSEDTAVYYCARGGPYFDYWGQGTLVTVSSASTKGPSVFPLAPSSKSTSGGTAALGCLVKDYFPEPVTVSWNSGALTSGVHTFPAVLQSSGLYSLSSVVTVPSSSLGTQTYICNVNHKPSNTKVDKKVEPKSCDKTHTCPPCPAPEAAGGPSVFLFPPKPKDTLMISRTPEVTCVVVDVSHEDPEVKFNWYVDGVEVHNAKTKPREEQYNSTYRVVSVLTVLHQDWLNGKEYKCKVSNKALPAPIEKTISKAKGQPREPQVYTLPPCREEMTKNQVSLWCLVKGFYPSDIAVEWESNGQPENNYKTTPPVLDSDGSFFLYSKLTVDKSRWQQGNVFSCSVMHEALHNHYTQKSLSLSPGK

SEQ ID NO: 228 - protein, 497 aa, Artificial Sequence
  PR004160 Chain
EVQLVESGGGVVQPGGSLRLSCAASGFTFSNYAMTWVRQAPEKGLEWVSSISGSGVSTYYADSVKGRFTISRDNSKNTLYLQMTRLTAEDTAVYFCAKEGSSETDDHYYNVDVWGQGTTVTVSSGGGGSGGGGSGGGGSEVQLVESGGGVVQPGGSLRLSCAASGFTFSNYAMTWVRQAPEKGLEWVSSISGSGVSTYYADSVKGRFTISRDNSKNTLYLQMTRLTAEDTAVYFCAKEGSSETDDHYYNVDVWGQGTTVTVSSASEPKSSDKTHTCPPCPAPEAAGGPSVFLFPPKPKDTLMISRTPEVTCVVVDVSHEDPEVKFNWYVDGVEVHNAKTKPREEQYNSTYRVVSVLTVLHQDWLNGKEYKCKVSNKALPAPIEKTISKAKGQPREPQVCTLPPSREEMTKNQVSLSCAVKGFYPSDIAVEWESNGQPENNYKTTPPVLDSDGSFFLVSKLTVDKSRWQQGNVFSCSVMHEALHNHYTQKSLSLSPGK

SEQ ID NO: 229 - protein, 638 aa, Artificial Sequence
  PR004161 Chain
EVQLVESGGGVVQPGGSLRLSCAASGFTFSNYAMTWVRQAPEKGLEWVSSISGSGVSTYYADSVKGRFTISRDNSKNTLYLQMTRLTAEDTAVYFCAKEGSSETDDHYYNVDVWGQGTTVTVSSGGGGSGGGGSGGGGSEVQLVESGGGVVQPGGSLRLSCAASGFTFSNYAMTWVRQAPEKGLEWVSSISGSGVSTYYADSVKGRFTISRDNSKNTLYLQMTRLTAEDTAVYFCAKEGSSETDDHYYNVDVWGQGTTVTVSSASGGGGSGGGGSGGGGSEVQLVESGGGVVQPGGSLRLSCAASGFTFSNYAMTWVRQAPEKGLEWVSSISGSGVSTYYADSVKGRFTISRDNSKNTLYLQMTRLTAEDTAVYFCAKEGSSETDDHYYNVDVWGQGTTVTVSSASEPKSSDKTHTCPPCPAPEAAGGPSVFLFPPKPKDTLMISRTPEVTCVVVDVSHEDPEVKFNWYVDGVEVHNAKTKPREEQYNSTYRVVSVLTVLHQDWLNGKEYKCKVSNKALPAPIEKTISKAKGQPREPQVCTLPPSREEMTKNQVSLSCAVKGFYPSDIAVEWESNGQPENNYKTTPPVLDSDGSFFLVSKLTVDKSRWQQGNVFSCSVMHEALHNHYTQKSLSLSPGK

SEQ ID NO: 230 - protein, 586 aa, Artificial Sequence
  PR004162 Chain
QVQLVQSGAEVKKPGSSMRVSCKASEDTFSSYAISWVRQAPGQGLEWMGGTAPIFGTTNYAQKFQGRVTITADKSTSTAYMELSSLRSEDTAVYYCARGGPYFDYWGQGTLVTVSSASTKGPSVFPLAPSSKSTSGGTAALGCLVKDYFPEPVTVSWNSGALTSGVHTFPAVLQSSGLYSLSSVVTVPSSSLGTQTYICNVNHKPSNTKVDKKVEPKSCDKTHTCPPCPAPEAAGGPSVFLFPPKPKDTLMISRTPEVTCVVVDVSHEDPEVKFNWYVDGVEVHNAKTKPREEQYNSTYRVVSVLTVLHQDWLNGKEYKCKVSNKALPAPIEKTISKAKGQPREPQVYTLPPSREEMTKNQVSLTCLVKGFYPSDIAVEWESNGQPENNYKTTPPVLDSDGSFFLYSKLTVDKSRWQQGNVFSCSVMHEALHNHYTQKSLSLSPGEPKSSDKTHTPPPPPRTEVQLVESGGGVVQPGGSLRLSCAASGFTFSNYAMTWVRQAPEKGLEWVSSISGSGVSTYYADSVKGRFTISRDNSKNTLYLQMTRLTAEDTAVYFCAKEGSSETDDHYYNVDVWGQGTTVTVSS

SEQ ID NO: 231 - protein, 636 aa, Artificial Sequence
  PR004181 Chain
EVQLLESGGGLVQPGGSLRLSCAASGFTFSNYAMTWVRQPPGKGLEWVSSISGSGGSTYYADSVKGRFTISRDNSKNTLYLQMNSLRAEDTAVYYCAKEGTGTTSDYYYNVDVWGQGTTVTVSSGGGGSGGGGSGGGGSEVQLLESGGGLVQPGGSLRLSCAASGFTFSNYAMTWVRQPPGKGLEWVSSISGSGGSTYYADSVKGRFTISRDNSKNTLYLQMNSLRAEDTAVYYCAKEGTGTTSDYYYNVDVWGQGTTVTVSSGGGGSGGGGSGGGGSEVQLLESGGGLVQPGGSLRLSCAASGFTFSNYAMTWVRQPPGKGLEWVSSISGSGGSTYYADSVKGRFTISRDNSKNTLYLQMNSLRAEDTAVYYCAKEGTGTTSDYYYNVDVWGQGTTVTVSSASEPKSSDKTHTCPPCPAPEAAGGPSVFLFPPKPKDTLMISRTPEVTCVVVDVSHEDPEVKFNWYVDGVEVHNAKTKPREEQYNSTYRVVSVLTVLHQDWLNGKEYKCKVSNKALPAPIEKTISKAKGQPREPQVCTLPPSREEMTKNQVSLSCAVKGFYPSDIAVEWESNGQPENNYKTTPPVLDSDGSFFLVSKLTVDKSRWQQGNVFSCSVMHEALHNHYTQKSLSLSPGK

SEQ ID NO: 232 - protein, 633 aa, Artificial Sequence
  PR004182 Chain
EVQLVESGGGLVQPGGSLRLSCAASGFTFSSYWMHWVRQAPGKGLVWVSRINSDGSSTSYADSVQGRFTISRDNAKNTLYLQMNSLRAEDTAVYYCVRKGSSSYYHYSIEDDWGQGTLVTVSSGGGGSGGGGSGGGGSEVQLVESGGGLVQPGGSLRLSCAASGFTFSSYWMHWVRQAPGKGLVWVSRINSDGSSTSYADSVQGRFTISRDNAKNTLYLQMNSLRAEDTAVYYCVRKGSSSYYHYSIEDDWGQGTLVTVSSGGGGSGGGGSGGGGSEVQLVESGGGLVQPGGSLRLSCAASGFTFSSYWMHWVRQAPGKGLVWVSRINSDGSSTSYADSVQGRFTISRDNAKNTLYLQMNSLRAEDTAVYYCVRKGSSSYYHYSIEDDWGQGTLVTVSSASEPKSSDKTHTCPPCPAPEAAGGPSVFLFPPKPKDTLMISRTPEVTCVVVDVSHEDPEVKFNWYVDGVEVHNAKTKPREEQYNSTYRVVSVLTVLHQDWLNGKEYKCKVSNKALPAPIEKTISKAKGQPREPQVCTLPPSREEMTKNQVSLSCAVKGFYPSDIAVEWESNGQPENNYKTTPPVLDSDGSFFLVSKLTVDKSRWQQGNVFSCSVMHEALHNHYTQKSLSLSPGK

SEQ ID NO: 233 - protein, 222 aa, Artificial Sequence
  PR004279 Chain, PR005189 Chain, PR005190 Chain, PR005649 Chain, PR0056
QVQLVESGGGVVQPGRSLRLSCAASGFTFRSFGMHWVRQAPGKGLEWVAVISYDASNEYYADSVKGRFIISRDNSKDTLYLQMNSLRAGDTAVYYCAKGGGLRWYFAYWGQGTLVTVSSASTKGPSVFPLAPSSKSTSGGTAALGCLVKDYFPEPVTVSWNSGALTSGVHTFPAVLQSSGLYSLSSVVTVPSSSLGTQTYICNVNHKPSNTKVDKKVEPKSC

SEQ ID NO: 234 - protein, 586 aa, Artificial Sequence
  PR004279 Chain
EIVMTQSPATLSVSPGERATLSCRASQSISSNLGWYQQKPGQAPRLLIYGASTRATGIPARFSGSGSGTEFTLTISSLQSEDFAVYYCQQYQSWPPLTFGGGTKVEIKRTVAAPSVFIFPPSDEQLKSGTASVVCLLNNFYPREAKVQWKVDNALQSGNSQESVTEQDSKDSTYSLSSTLTLSKADYEKHKVYACEVTHQGLSSPVTKSFNRGECEPKSSDKTHTPPPPPEVQLVESGGGVVQPGGSLRLSCAASGFTFSNYAMTWVRQAPEKGLEWVSSISGSGVSTYYADSVKGRFTISRDNSKNTLYLQMTRLTAEDTAVYFCAKEGSSETDDHYYNVDVWGQGTTVTVSSEPKSSDKTHTCPPCPAPEAAGGPSVFLFPPKPKDTLMISRTPEVTCVVVDVSHEDPEVKFNWYVDGVEVHNAKTKPREEQYNSTYRVVSVLTVLHQDWLNGKEYKCKVSNKALPAPIEKTISKAKGQPREPQVYTLPPSREEMTKNQVSLTCLVKGFYPSDIAVEWESNGQPENNYKTTPPVLDSDGSFFLYSKLTVDKSRWQQGNVFSCSVMHEALHNHYTQKSLSLSPGK

SEQ ID NO: 235 - protein, 578 aa, Artificial Sequence
  PR004280 Chain
QVQLVESGGGVVQPGRSLRLSCAASGFTFRSFGMHWVRQAPGKGLEWVAVISYDASNEYYADSVKGRFIISRDNSKDTLYLQMNSLRAGDTAVYYCAKGGGLRWYFAYWGQGTLVTVSSASTKGPSVFPLAPSSKSTSGGTAALGCLVKDYFPEPVTVSWNSGALTSGVHTFPAVLQSSGLYSLSSVVTVPSSSLGTQTYICNVNHKPSNTKVDKKVEPKSCDKTHTCPPCPAPEAAGGPSVFLFPPKPKDTLMISRTPEVTCVVVDVSHEDPEVKFNWYVDGVEVHNAKTKPREEQYNSTYRVVSVLTVLHQDWLNGKEYKCKVSNKALPAPIEKTISKAKGQPREPQVYTLPPSREEMTKNQVSLTCLVKGFYPSDIAVEWESNGQPENNYKTTPPVLDSDGSFFLYSKLTVDKSRWQQGNVFSCSVMHEALHNHYTQKSLSLSPGEPKSSDEVQLLESGGGLVQPGGSLRLSCAASGFTFSNYAMSWFRQPPETGLKWVSSIDASGGDTYYADSVKGRFTISRDNSKNTLYLQMNSLRAEDTAVYYCAKEGSHGTDDSHYDVDVWGQGTTVTVSS

SEQ ID NO: 236 - protein, 572 aa, Artificial Sequence
  PR004281 Chain
QVQLVESGGGVVQPGRSLRLSCAASGFTFRSFGMHWVRQAPGKGLEWVAVISYDASNEYYADSVKGRFIISRDNSKDTLYLQMNSLRAGDTAVYYCAKGGGLRWYFAYWGQGTLVTVSSASTKGPSVFPLAPSSKSTSGGTAALGCLVKDYFPEPVTVSWNSGALTSGVHTFPAVLQSSGLYSLSSVVTVPSSSLGTQTYICNVNHKPSNTKVDKKVEPKSCDKTHTCPPCPAPEAAGGPSVFLFPPKPKDTLMISRTPEVTCVVVDVSHEDPEVKFNWYVDGVEVHNAKTKPREEQYNSTYRVVSVLTVLHQDWLNGKEYKCKVSNKALPAPIEKTISKAKGQPREPQVYTLPPSREEMTKNQVSLTCLVKGFYPSDIAVEWESNGQPENNYKTTPPVLDSDGSFFLYSKLTVDKSRWQQGNVFSCSVMHEALHNHYTQKSLSLSPGEVQLLESGGGLVQPGGSLRLSCAASGFTFSNYAMSWFRQPPETGLKWVSSIDASGGDTYYADSVKGRFTISRDNSKNTLYLQMNSLRAEDTAVYYCAKEGSHGTDDSHYDVDVWGQGTTVTVSS

SEQ ID NO: 237 - protein, 578 aa, Artificial Sequence
  PR004282 Chain
QVQLVESGGGVVQPGRSLRLSCAASGFTFRSFGMHWVRQAPGKGLEWVAVISYDASNEYYADSVKGRFIISRDNSKDTLYLQMNSLRAGDTAVYYCAKGGGLRWYFAYWGQGTLVTVSSASTKGPSVFPLAPSSKSTSGGTAALGCLVKDYFPEPVTVSWNSGALTSGVHTFPAVLQSSGLYSLSSVVTVPSSSLGTQTYICNVNHKPSNTKVDKKVEPKSCDKTHTCPPCPAPEAAGGPSVFLFPPKPKDTLMISRTPEVTCVVVDVSHEDPEVKFNWYVDGVEVHNAKTKPREEQYNSTYRVVSVLTVLHQDWLNGKEYKCKVSNKALPAPIEKTISKAKGQPREPQVYTLPPSREEMTKNQVSLTCLVKGFYPSDIAVEWESNGQPENNYKTTPPVLDSDGSFFLYSKLTVDKSRWQQGNVFSCSVMHEALHNHYTQKSLSLSPGGGSGGSEVQLLESGGGLVQPGGSLRLSCAASGFTFSNYAMSWFRQPPETGLKWVSSIDASGGDTYYADSVKGRFTISRDNSKNTLYLQMNSLRAEDTAVYYCAKEGSHGTDDSHYDVDVWGQGTTVTVSS

SEQ ID NO: 238 - protein, 585 aa, Artificial Sequence
  PR004357 Chain
QVQLVQSGAEVKKPGSSMRVSCKASEDTFSSYAISWVRQAPGQGLEWMGGTAPIFGTTNYAQKFQGRVTITADKSTSTAYMELSSLRSEDTAVYYCARGGPYFDYWGQGTLVTVSSASTKGPSVFPLAPSSKSTSGGTAALGCLVKDYFPEPVTVSWNSGALTSGVHTFPAVLQSSGLYSLSSVVTVPSSSLGTQTYICNVNHKPSNTKVDKKVEPKSCDKTHTCPPCPAPEAAGGPSVFLFPPKPKDTLMISRTPEVTCVVVDVSHEDPEVKFNWYVDGVEVHNAKTKPREEQYNSTYRVVSVLTVLHQDWLNGKEYKCKVSNKALGAPIEKTISKAKGQPREPQVYTLPPSREEMTKNQVSLTCLVKGFYPSDIAVEWESNGQPENNYKTTPPVLDSDGSFFLYSKLTVDKSRWQQGNVFSCSVMHEALHNHYTQKSLSLSPGEPKSSDKTHTPPPPPRTEVQLVESGGGLVQPGGSLRLSCAASGFTFSSYWMHWVRQAPGKGLVWVSRINSDGSSTSYADSVQGRFTISRDNAKNTLYLQMNSLRAEDTAVYYCVRKGSSSYYHYSIEDDWGQGTLVTVSS

SEQ ID NO: 239 - protein, 713 aa, Artificial Sequence
  PR004358 Chain
QVQLVQSGAEVKKPGSSMRVSCKASEDTFSSYAISWVRQAPGQGLEWMGGTAPIFGTTNYAQKFQGRVTITADKSTSTAYMELSSLRSEDTAVYYCARGGPYFDYWGQGTLVTVSSASTKGPSVFPLAPSSKSTSGGTAALGCLVKDYFPEPVTVSWNSGALTSGVHTFPAVLQSSGLYSLSSVVTVPSSSLGTQTYICNVNHKPSNTKVDKKVEPKSCDKTHTCPPCPAPEAAGGPSVFLFPPKPKDTLMISRTPEVTCVVVDVSHEDPEVKFNWYVDGVEVHNAKTKPREEQYNSTYRVVSVLTVLHQDWLNGKEYKCKVSNKALGAPIEKTISKAKGQPREPQVYTLPPSREEMTKNQVSLTCLVKGFYPSDIAVEWESNGQPENNYKTTPPVLDSDGSFFLYSKLTVDKSRWQQGNVFSCSVMHEALHNHYTQKSLSLSPGEPKSSDKTHTPPPPPRTEVQLVESGGGLVQPGGSLRLSCAASGFTFSSYWMHWVRQAPGKGLVWVSRINSDGSSTSYADSVQGRFTISRDNAKNTLYLQMNSLRAEDTAVYYCVRKGSSSYYHYSIEDDWGQGTLVTVSSGGGGSEVQLVESGGGLVQPGGSLRLSCAASGFTFSSYWMHWVRQAPGKGLVWVSRINSDGSSTSYADSVQGRFTISRDNAKNTLYLQMNSLRAEDTAVYYCVRKGSSSYYHYSIEDDWGQGTLVTVSS

SEQ ID NO: 240 - protein, 586 aa, Artificial Sequence
  PR004359 Chain
QVQLVQSGAEVKKPGSSMRVSCKASEDTFSSYAISWVRQAPGQGLEWMGGTAPIFGTTNYAQKFQGRVTITADKSTSTAYMELSSLRSEDTAVYYCARGGPYFDYWGQGTLVTVSSASTKGPSVFPLAPSSKSTSGGTAALGCLVKDYFPEPVTVSWNSGALTSGVHTFPAVLQSSGLYSLSSVVTVPSSSLGTQTYICNVNHKPSNTKVDKKVEPKSCDKTHTCPPCPAPEAAGGPSVFLFPPKPKDTLMISRTPEVTCVVVDVSHEDPEVKFNWYVDGVEVHNAKTKPREEQYNSTYRVVSVLTVLHQDWLNGKEYKCKVSNKALPAPIEKTISKAKGQPREPQVYTLPPSREEMTKNQVSLTCLVKGFYPSDIAVEWESNGQPENNYKTTPPVLDSDGSFFLYSKLTVDKSRWQQGNVFSCSVMHEALHNHYTQKSLSLSPGEPKSSDKTHTPPPPPRTEVQLLESGGGLVQPGGSLRLSCAASGFTFSNYAMSWFRQPPETGLKWVSSIDGSGGDTYYADSVKGRFTISRDNSKNTLYLQMNSLRAEDTAVYYCAKEGSHGTDDSHYDVDVWGQGTTVTVSS

SEQ ID NO: 241 - protein, 4 aa, Artificial Sequence
  GS_4
GSGS

SEQ ID NO: 242 - protein, 5 aa, Artificial Sequence
  GS_5
GGGGS

SEQ ID NO: 243 - protein, 6 aa, Artificial Sequence
  GS_6
GGSGGS

SEQ ID NO: 244 - protein, 7 aa, Artificial Sequence
  GS_7
GGGGSGS

SEQ ID NO: 245 - protein, 15 aa, Artificial Sequence
  GS_15
GGGGSGGGGSGGGGS

SEQ ID NO: 246 - protein, 20 aa, Artificial Sequence
  GS_20
GGGGSGGGGSGGGGSGGGGS

SEQ ID NO: 247 - protein, 25 aa, Artificial Sequence
  GS_25
GGGGSGGGGSGGGGSGGGGSGGGGS

SEQ ID NO: 248 - protein, 15 aa, Artificial Sequence
  human IgG1 hinge
EPKSCDKTHTCPPCP

SEQ ID NO: 249 - protein, 15 aa, Artificial Sequence
  human IgG1 hinge (C220S)
EPKSSDKTHTCPPCP

SEQ ID NO: 250 - protein, 15 aa, Artificial Sequence
  H1_15
EPKSSDKTHTPPPPP

SEQ ID NO: 251 - protein, 15 aa, Artificial Sequence
  G5-LH
GGGGGDKTHTCPPCP

SEQ ID NO: 252 - protein, 17 aa, Artificial Sequence
  H1_15-RT
EPKSSDKTHTPPPPPRT

SEQ ID NO: 253 - protein, 18 aa, Artificial Sequence
  L-GS_15-RT
LGGGGSGGGGSGGGGSRT

SEQ ID NO: 254 - protein, 18 aa, Artificial Sequence
  L-H1_15-RT
LEPKSSDKTHTPPPPPRT

SEQ ID NO: 255 - protein, 19 aa, Artificial Sequence
  KL-H1_15-RT
KLEPKSSDKTHTPPPPPRT

SEQ ID NO: 256 - protein, 19 aa, Artificial Sequence
  KL-H1_15-AS
KLEPKSSDKTHTPPPPPAS

SEQ ID NO: 257 - protein, 9 aa, Artificial Sequence
  RT-GS_5-KL
RTGGGGSKL

SEQ ID NO: 258 - protein, 19 aa, Artificial Sequence
  RT-GS_15-KL
RTGGGGSGGGGSGGGGSKL

SEQ ID NO: 259 - protein, 29 aa, Artificial Sequence
  RT-GS_25-KL
RTGGGGSGGGGSGGGGSGGGGSGGGGSKL

SEQ ID NO: 260 - protein, 6 aa, Artificial Sequence
  EPKSSD
EPKSSD

SEQ ID NO: 261 - protein, 17 aa, Artificial Sequence
  AS-GS_15
ASGGGGSGGGGSGGGGS

SEQ ID NO: 262 - protein, 569 aa, Artificial Sequence
  PR004995 Chain
QVQLVQSGAEVKKPGSSMRVSCKASEDTFSSYAISWVRQAPGQGLEWMGGTAPIFGTTNYAQKFQGRVTITADKSTSTAYMELSSLRSEDTAVYYCARGGPYFDYWGQGTLVTVSSASTKGPSVFPLAPSSKSTSGGTAALGCLVKDYFPEPVTVSWNSGALTSGVHTFPAVLQSSGLYSLSSVVTVPSSSLGTQTYICNVNHKPSNTKVDKKVEPKSCDKTHTCPPCPAPEAAGGPSVFLFPPKPKDTLMISRTPEVTCVVVDVSHEDPEVKFNWYVDGVEVHNAKTKPREEQYNSTYRVVSVLTVLHQDWLNGKEYKCKVSNKALPAPIEKTISKAKGQPREPQVYTLPPSREEMTKNQVSLTCLVKGFYPSDIAVEWESNGQPENNYKTTPPVLDSDGSFFLYSKLTVDKSRWQQGNVFSCSVMHEALHNHYTQKSLSLSPGEVQLLESGGGLVQPGGSLRLSCAASGFTFSNYAMSWFRQPPETGLKWVSSIDASGGDTYYADSVKGRFTISRDNSKNTLYLQMNSLRAEDTAVYYCAKEGSHGTDDSHYDVDVWGQGTTVTVSS

SEQ ID NO: 263 - protein, 572 aa, Artificial Sequence
  PR005183 Chain
QVQLVESGGGVVQPGRSLRLSCAASGFTFRSFGMHWVRQAPGKGLEWVAVISYDASNEYYADSVKGRFIISRDNSKDTLYLQMNSLRAGDTAVYYCAKGGGLRWYFAYWGQGTLVTVSSASTKGPSVFPLAPSSKSTSGGTAALGCLVKDYFPEPVTVSWNSGALTSGVHTFPAVLQSSGLYSLSSVVTVPSSSLGTQTYICNVNHKPSNTKVDKKVEPKSCDKTHTCPPCPAPEAAGGPSVFLFPPKPKDTLMISRTPEVTCVVVDVSHEDPEVKFNWYVDGVEVHNAKTKPREEQYNSTYRVVSVLTVLHQDWLNGKEYKCKVSNKALGAPIEKTISKAKGQPREPQVYTLPPSREEMTKNQVSLTCLVKGFYPSDIAVEWESNGQPENNYKTTPPVLDSDGSFFLYSKLTVDKSRWQQGNVFSCSVMHEALHNHYTQKSLSLSPGEVQLLESGGGLVQPGGSLRLSCAASGFTFSNYAMSWFRQPPETGLKWVSSIDASGGDTYYADSVKGRFTISRDNSKNTLYLQMNSLRAEDTAVYYCAKEGSHGTDDSHYDVDVWGQGTTVTVSS

SEQ ID NO: 264 - protein, 569 aa, Artificial Sequence
  PR005184 Chain
QVQLVESGGGVVQPGRSLRLSCAASGFTFRSFGMHWVRQAPGKGLEWVAVISYDASNEYYADSVKGRFIISRDNSKDTLYLQMNSLRAGDTAVYYCAKGGGLRWYFAYWGQGTLVTVSSASTKGPSVFPLAPSSKSTSGGTAALGCLVKDYFPEPVTVSWNSGALTSGVHTFPAVLQSSGLYSLSSVVTVPSSSLGTQTYICNVNHKPSNTKVDKKVEPKSCDKTHTCPPCPAPGGPSVFLFPPKPKDTLMISRTPEVTCVVVDVSHEDPEVKFNWYVDGVEVHNAKTKPREEQYNSTYRVVSVLTVLHQDWLNGKEYKCKVSNKALPAPIEKTISKAKGQPREPQVYTLPPSREEMTKNQVSLTCLVKGFYPSDIAVEWESNGQPENNYKTTPPVLDSDGSFFLYSKLTVDKSRWQQGNVFSCSVMHEALHNHYTQKSLSLSPGEVQLLESGGGLVQPGGSLRLSCAASGFTFSNYAMSWFRQPPETGLKWVSSIDASGGDTYYADSVKGRFTISRDNSKNTLYLQMNSLRAEDTAVYYCAKEGSHGTDDSHYDVDVWGQGTTVTVSS

SEQ ID NO: 265 - protein, 569 aa, Artificial Sequence
  PR005185 Chain
QVQLVESGGGVVQPGRSLRLSCAASGFTFRSFGMHWVRQAPGKGLEWVAVISYDASNEYYADSVKGRFIISRDNSKDTLYLQMNSLRAGDTAVYYCAKGGGLRWYFAYWGQGTLVTVSSASTKGPSVFPLAPCSRSTSESTAALGCLVKDYFPEPVTVSWNSGALTSGVHTFPAVLQSSGLYSLSSVVTVPSSSLGTKTYTCNVDHKPSNTKVDKRVESKYGPPCPPCPAPEAAGGPSVFLFPPKPKDTLMISRTPEVTCVVVDVSQEDPEVQFNWYVDGVEVHNAKTKPREEQFNSTYRVVSVLTVLHQDWLNGKEYKCKVSNKGLPSSIEKTISKAKGQPREPQVYTLPPSQEEMTKNQVSLTCLVKGFYPSDIAVEWESNGQPENNYKTTPPVLDSDGSFFLYSRLTVDKSRWQEGNVFSCSVMHEALHNHYTQKSLSLSLGEVQLLESGGGLVQPGGSLRLSCAASGFTFSNYAMSWFRQPPETGLKWVSSIDASGGDTYYADSVKGRFTISRDNSKNTLYLQMNSLRAEDTAVYYCAKEGSHGTDDSHYDVDVWGQGTTVTVSS

SEQ ID NO: 266 - protein, 572 aa, Artificial Sequence
  PR005186 Chain
QVQLVESGGGVVQPGRSLRLSCAASGFTFRSFGMHWVRQAPGKGLEWVAVISYDASNEYYADSVKGRFIISRDNSKDTLYLQMNSLRAGDTAVYYCAKGGGLRWYFAYWGQGTLVTVSSASTKGPSVFPLAPSSKSTSGGTAALGCLVKDYFPEPVTVSWNSGALTSGVHTFPAVLQSSGLYSLSSVVTVPSSSLGTQTYICNVNHKPSNTKVDKKVEPKSCDKTHTCPPCPAPELAGAPSVFLFPPKPKDTLMISRTPEVTCVVVDVSHEDPEVKFNWYVDGVEVHNAKTKPREEQYNSTYRVVSVLTVLHQDWLNGKEYKCKVSNKALPAPIEKTISKAKGQPREPQVYTLPPSREEMTKNQVSLTCLVKGFYPSDIAVEWESNGQPENNYKTTPPVLDSDGSFFLYSKLTVDKSRWQQGNVFSCSVMHEALHNHYTQKSLSLSPGEVQLLESGGGLVQPGGSLRLSCAASGFTFSNYAMSWFRQPPETGLKWVSSIDASGGDTYYADSVKGRFTISRDNSKNTLYLQMNSLRAEDTAVYYCAKEGSHGTDDSHYDVDVWGQGTTVTVSS

SEQ ID NO: 267 - protein, 572 aa, Artificial Sequence
  PR005187 Chain
QVQLVESGGGVVQPGRSLRLSCAASGFTFRSFGMHWVRQAPGKGLEWVAVISYDASNEYYADSVKGRFIISRDNSKDTLYLQMNSLRAGDTAVYYCAKGGGLRWYFAYWGQGTLVTVSSASTKGPSVFPLAPSSKSTSGGTAALGCLVKDYFPEPVTVSWNSGALTSGVHTFPAVLQSSGLYSLSSVVTVPSSSLGTQTYICNVNHKPSNTKVDKKVEPKSCDKTHTCPPCPAPEAAGGPSVFLFPPKPKDTLYITREPEVTCVVVDVSHEDPEVKFNWYVDGVEVHNAKTKPREEQYNSTYRVVSVLTVLHQDWLNGKEYKCKVSNKALPAPIEKTISKAKGQPREPQVYTLPPSREEMTKNQVSLTCLVKGFYPSDIAVEWESNGQPENNYKTTPPVLDSDGSFFLYSKLTVDKSRWQQGNVFSCSVMHEALHNHYTQKSLSLSPGEVQLLESGGGLVQPGGSLRLSCAASGFTFSNYAMSWFRQPPETGLKWVSSIDASGGDTYYADSVKGRFTISRDNSKNTLYLQMNSLRAEDTAVYYCAKEGSHGTDDSHYDVDVWGQGTTVTVSS

SEQ ID NO: 268 - protein, 572 aa, Artificial Sequence
  PR005188 Chain
QVQLVESGGGVVQPGRSLRLSCAASGFTFRSFGMHWVRQAPGKGLEWVAVISYDASNEYYADSVKGRFIISRDNSKDTLYLQMNSLRAGDTAVYYCAKGGGLRWYFAYWGQGTLVTVSSASTKGPSVFPLAPSSKSTSGGTAALGCLVKDYFPEPVTVSWNSGALTSGVHTFPAVLQSSGLYSLSSVVTVPSSSLGTQTYICNVNHKPSNTKVDKKVEPKSCDKTHTCPPCPAPEAAGGPSVFLFPPKPKDTLMISRTPEVTCVVVDVSHEDPEVKFNWYVDGVEVHNAKTKPREEQYNSTYRVVSVLTVDHHDWLNGKEYKCKVSNKALPAPIEKTISKAKGQPREPQVYTLPPSREEMTKNQVSLTCLVKGFYPSDIAVEWESNGQPENNYKTTPPVLDSDGSFFLYSKLTVDKSRWQQGNVFSCSVMHEALHSHYTQKSLSLSPGEVQLLESGGGLVQPGGSLRLSCAASGFTFSNYAMSWFRQPPETGLKWVSSIDASGGDTYYADSVKGRFTISRDNSKNTLYLQMNSLRAEDTAVYYCAKEGSHGTDDSHYDVDVWGQGTTVTVSS

SEQ ID NO: 269 - protein, 571 aa, Artificial Sequence
  PR005189 Chain
EIVMTQSPATLSVSPGERATLSCRASQSISSNLGWYQQKPGQAPRLLIYGASTRATGIPARFSGSGSGTEFTLTISSLQSEDFAVYYCQQYQSWPPLTFGGGTKVEIKRTVAAPSVFIFPPSDEQLKSGTASVVCLLNNFYPREAKVQWKVDNALQSGNSQESVTEQDSKDSTYSLSSTLTLSKADYEKHKVYACEVTHQGLSSPVTKSFNRGECEVQLVESGGGVVQPGGSLRLSCAASGFTFSNYAMTWVRQAPEKGLEWVSSISGSGVSTYYADSVKGRFTISRDNSKNTLYLQMTRLTAEDTAVYFCAKEGSSETDDHYYNVDVWGQGTTVTVSSEPKSSDKTHTCPPCPAPEAAGGPSVFLFPPKPKDTLMISRTPEVTCVVVDVSHEDPEVKFNWYVDGVEVHNAKTKPREEQYNSTYRVVSVLTVLHQDWLNGKEYKCKVSNKALPAPIEKTISKAKGQPREPQVYTLPPSREEMTKNQVSLTCLVKGFYPSDIAVEWESNGQPENNYKTTPPVLDSDGSFFLYSKLTVDKSRWQQGNVFSCSVMHEALHNHYTQKSLSLSPGK

SEQ ID NO: 270 - protein, 571 aa, Artificial Sequence
  PR005190 Chain
EIVMTQSPATLSVSPGERATLSCRASQSISSNLGWYQQKPGQAPRLLIYGASTRATGIPARFSGSGSGTEFTLTISSLQSEDFAVYYCQQYQSWPPLTFGGGTKVEIKRTVAAPSVFIFPPSDEQLKSGTASVVCLLNNFYPREAKVQWKVDNALQSGNSQESVTEQDSKDSTYSLSSTLTLSKADYEKHKVYACEVTHQGLSSPVTKSFNRGECEVQLLESGGGLVQPGGSLRLSCAASGFTFSNYAMSWFRQPPETGLKWVSSIDASGGDTYYADSVKGRFTISRDNSKNTLYLQMNSLRAEDTAVYYCAKEGSHGTDDSHYDVDVWGQGTTVTVSSEPKSSDKTHTCPPCPAPEAAGGPSVFLFPPKPKDTLMISRTPEVTCVVVDVSHEDPEVKFNWYVDGVEVHNAKTKPREEQYNSTYRVVSVLTVLHQDWLNGKEYKCKVSNKALPAPIEKTISKAKGQPREPQVYTLPPSREEMTKNQVSLTCLVKGFYPSDIAVEWESNGQPENNYKTTPPVLDSDGSFFLYSKLTVDKSRWQQGNVFSCSVMHEALHNHYTQKSLSLSPGK

SEQ ID NO: 271 - protein, 583 aa, Artificial Sequence
  PR005649 Chain
EIVMTQSPATLSVSPGERATLSCRASQSISSNLGWYQQKPGQAPRLLIYGASTRATGIPARFSGSGSGTEFTLTISSLQSEDFAVYYCQQYQSWPPLTFGGGTKVEIKRTVAAPSVFIFPPSDEQLKSGTASVVCLLNNFYPREAKVQWKVDNALQSGNSQESVTEQDSKDSTYSLSSTLTLSKADYEKHKVYACEVTHQGLSSPVTKSFNRGECEPKSSDKTHTPPPPPEVQLVESGGGVVQPGGSLRLSCAASGFTFSNYAMTWVRQAPEKGLEWVSSISGSGVSTYYADSVKGRFTISRDNSKNTLYLQMTRLTAEDTAVYFCAKEGSSETDDHYYNVDVWGQGTTVTVSSERKCCVECPPCPAPEAAGGPSVFLFPPKPKDTLMISRTPEVTCVVVDVSHEDPEVKFNWYVDGVEVHNAKTKPREEQYNSTYRVVSVLTVLHQDWLNGKEYKCKVSNKALPAPIEKTISKAKGQPREPQVYTLPPSREEMTKNQVSLTCLVKGFYPSDIAVEWESNGQPENNYKTTPPVLDSDGSFFLYSKLTVDKSRWQQGNVFSCSVMHEALHNHYTQKSLSLSPGK

SEQ ID NO: 272 - protein, 694 aa, Artificial Sequence
  PR005650 Chain
EIVMTQSPATLSVSPGERATLSCRASQSISSNLGWYQQKPGQAPRLLIYGASTRATGIPARFSGSGSGTEFTLTISSLQSEDFAVYYCQQYQSWPPLTFGGGTKVEIKRTVAAPSVFIFPPSDEQLKSGTASVVCLLNNFYPREAKVQWKVDNALQSGNSQESVTEQDSKDSTYSLSSTLTLSKADYEKHKVYACEVTHQGLSSPVTKSFNRGECEVQLVESGGGVVQPGGSLRLSCAASGFTFSNYAMTWVRQAPEKGLEWVSSISGSGVSTYYADSVKGRFTISRDNSKNTLYLQMTRLTAEDTAVYFCAKEGSSETDDHYYNVDVWGQGTTVTVSSEPKSSDKTHTCPPCPAPEAAGGPSVFLFPPKPKDTLMISRTPEVTCVVVDVSHEDPEVKFNWYVDGVEVHNAKTKPREEQYNSTYRVVSVLTVLHQDWLNGKEYKCKVSNKALPAPIEKTISKAKGQPREPQVYTLPPSREEMTKNQVSLTCLVKGFYPSDIAVEWESNGQPENNYKTTPPVLDSDGSFFLYSKLTVDKSRWQQGNVFSCSVMHEALHNHYTQKSLSLSPGEVQLVESGGGVVQPGGSLRLSCAASGFTFSNYAMTWVRQAPEKGLEWVSSISGSGVSTYYADSVKGRFTISRDNSKNTLYLQMTRLTAEDTAVYFCAKEGSSETDDHYYNVDVWGQGTTVTVSS

SEQ ID NO: 273 - protein, 694 aa, Artificial Sequence
  PR005651 Chain
EIVMTQSPATLSVSPGERATLSCRASQSISSNLGWYQQKPGQAPRLLIYGASTRATGIPARFSGSGSGTEFTLTISSLQSEDFAVYYCQQYQSWPPLTFGGGTKVEIKRTVAAPSVFIFPPSDEQLKSGTASVVCLLNNFYPREAKVQWKVDNALQSGNSQESVTEQDSKDSTYSLSSTLTLSKADYEKHKVYACEVTHQGLSSPVTKSFNRGECEVQLLESGGGLVQPGGSLRLSCAASGFTFSNYAMSWFRQPPETGLKWVSSIDASGGDTYYADSVKGRFTISRDNSKNTLYLQMNSLRAEDTAVYYCAKEGSHGTDDSHYDVDVWGQGTTVTVSSEPKSSDKTHTCPPCPAPEAAGGPSVFLFPPKPKDTLMISRTPEVTCVVVDVSHEDPEVKFNWYVDGVEVHNAKTKPREEQYNSTYRVVSVLTVLHQDWLNGKEYKCKVSNKALPAPIEKTISKAKGQPREPQVYTLPPSREEMTKNQVSLTCLVKGFYPSDIAVEWESNGQPENNYKTTPPVLDSDGSFFLYSKLTVDKSRWQQGNVFSCSVMHEALHNHYTQKSLSLSPGEVQLLESGGGLVQPGGSLRLSCAASGFTFSNYAMSWFRQPPETGLKWVSSIDASGGDTYYADSVKGRFTISRDNSKNTLYLQMNSLRAEDTAVYYCAKEGSHGTDDSHYDVDVWGQGTTVTVSS

SEQ ID NO: 274 - protein, 582 aa, Artificial Sequence
  PR005827 Chain
QVQLVESGGGVVQPGRSLRLSCAASGFTFRSFGMHWVRQAPGKGLEWVAVISYDASNEYYADSVKGRFIISRDNSKDTLYLQMNSLRAGDTAVYYCAKGGGLRWYFAYWGQGTLVTVSSASTKGPSVFPLAPSSKSTSGGTAALGCLVKDYFPEPVTVSWNSGALTSGVHTFPAVLQSSGLYSLSSVVTVPSSSLGTQTYICNVNHKPSNTKVDKKVEPKSCDKTHTCPPCPAPEAAGGPSVFLFPPKPKDTLMISRTPEVTCVVVDVSHEDPEVKFNWYVDGVEVHNAKTKPREEQYNSTYRVVSVLTVLHQDWLNGKEYKCKVSNKALPAPIEKTISKAKGQPREPQVYTLPPSREEMTKNQVSLTCLVKGFYPSDIAVEWESNGQPENNYKTTPPVLDSDGSFFLYSKLTVDKSRWQQGNVFSCSVMHEALHNHYTQKSLSLSPGGGGGSGGGGSEVQLLESGGGLVQPGGSLRLSCAASGFTFSNYAMSWFRQPPETGLKWVSSIDASGGDTYYADSVKGRFTISRDNSKNTLYLQMNSLRAEDTAVYYCAKEGSHGTDDSHYDVDVWGQGTTVTVSS

SEQ ID NO: 275 - protein, 587 aa, Artificial Sequence
  PR005828 Chain
QVQLVESGGGVVQPGRSLRLSCAASGFTFRSFGMHWVRQAPGKGLEWVAVISYDASNEYYADSVKGRFIISRDNSKDTLYLQMNSLRAGDTAVYYCAKGGGLRWYFAYWGQGTLVTVSSASTKGPSVFPLAPSSKSTSGGTAALGCLVKDYFPEPVTVSWNSGALTSGVHTFPAVLQSSGLYSLSSVVTVPSSSLGTQTYICNVNHKPSNTKVDKKVEPKSCDKTHTCPPCPAPEAAGGPSVFLFPPKPKDTLMISRTPEVTCVVVDVSHEDPEVKFNWYVDGVEVHNAKTKPREEQYNSTYRVVSVLTVLHQDWLNGKEYKCKVSNKALPAPIEKTISKAKGQPREPQVYTLPPSREEMTKNQVSLTCLVKGFYPSDIAVEWESNGQPENNYKTTPPVLDSDGSFFLYSKLTVDKSRWQQGNVFSCSVMHEALHNHYTQKSLSLSPGGGGGSGGGGSGGGGSEVQLLESGGGLVQPGGSLRLSCAASGFTFSNYAMSWFRQPPETGLKWVSSIDASGGDTYYADSVKGRFTISRDNSKNTLYLQMNSLRAEDTAVYYCAKEGSHGTDDSHYDVDVWGQGTTVTVSS

SEQ ID NO: 276 - protein, 592 aa, Artificial Sequence
  PR005829 Chain
QVQLVESGGGVVQPGRSLRLSCAASGFTFRSFGMHWVRQAPGKGLEWVAVISYDASNEYYADSVKGRFIISRDNSKDTLYLQMNSLRAGDTAVYYCAKGGGLRWYFAYWGQGTLVTVSSASTKGPSVFPLAPSSKSTSGGTAALGCLVKDYFPEPVTVSWNSGALTSGVHTFPAVLQSSGLYSLSSVVTVPSSSLGTQTYICNVNHKPSNTKVDKKVEPKSCDKTHTCPPCPAPEAAGGPSVFLFPPKPKDTLMISRTPEVTCVVVDVSHEDPEVKFNWYVDGVEVHNAKTKPREEQYNSTYRVVSVLTVLHQDWLNGKEYKCKVSNKALPAPIEKTISKAKGQPREPQVYTLPPSREEMTKNQVSLTCLVKGFYPSDIAVEWESNGQPENNYKTTPPVLDSDGSFFLYSKLTVDKSRWQQGNVFSCSVMHEALHNHYTQKSLSLSPGGGGGSGGGGSGGGGSGGGGSEVQLLESGGGLVQPGGSLRLSCAASGFTFSNYAMSWFRQPPETGLKWVSSIDASGGDTYYADSVKGRFTISRDNSKNTLYLQMNSLRAEDTAVYYCAKEGSHGTDDSHYDVDVWGQGTTVTVSS

SEQ ID NO: 277 - protein, 597 aa, Artificial Sequence
  PR005830 Chain
QVQLVESGGGVVQPGRSLRLSCAASGFTFRSFGMHWVRQAPGKGLEWVAVISYDASNEYYADSVKGRFIISRDNSKDTLYLQMNSLRAGDTAVYYCAKGGGLRWYFAYWGQGTLVTVSSASTKGPSVFPLAPSSKSTSGGTAALGCLVKDYFPEPVTVSWNSGALTSGVHTFPAVLQSSGLYSLSSVVTVPSSSLGTQTYICNVNHKPSNTKVDKKVEPKSCDKTHTCPPCPAPEAAGGPSVFLFPPKPKDTLMISRTPEVTCVVVDVSHEDPEVKFNWYVDGVEVHNAKTKPREEQYNSTYRVVSVLTVLHQDWLNGKEYKCKVSNKALPAPIEKTISKAKGQPREPQVYTLPPSREEMTKNQVSLTCLVKGFYPSDIAVEWESNGQPENNYKTTPPVLDSDGSFFLYSKLTVDKSRWQQGNVFSCSVMHEALHNHYTQKSLSLSPGGGGGSGGGGSGGGGSGGGGSGGGGSEVQLLESGGGLVQPGGSLRLSCAASGFTFSNYAMSWFRQPPETGLKWVSSIDASGGDTYYADSVKGRFTISRDNSKNTLYLQMNSLRAEDTAVYYCAKEGSHGTDDSHYDVDVWGQGTTVTVSS

SEQ ID NO: 278 - protein, 578 aa, Artificial Sequence
  PR005838 Chain
QVQLVESGGGVVQPGRSLRLSCAASGFTFRSFGMHWVRQAPGKGLEWVAVISYDASNEYYADSVKGRFIISRDNSKDTLYLQMNSLRAGDTAVYYCAKGGGLRWYFAYWGQGTLVTVSSASTKGPSVFPLAPSSKSTSGGTAALGCLVKDYFPEPVTVSWNSGALTSGVHTFPAVLQSSGLYSLSSVVTVPSSSLGTQTYICNVNHKPSNTKVDKKVEPKSCDKTHTCPPCPAPEAAGAPSVFLFPPKPKDTLMISRTPEVTCVVVDVSHEDPEVKFNWYVDGVEVHNAKTKPREEQYNSTYRVVSVLTVLHQDWLNGKEYKCKVSNKALPAPIEKTISKAKGQPREPQVYTLPPSREEMTKNQVSLTCLVKGFYPSDIAVEWESNGQPENNYKTTPPVLDSDGSFFLYSKLTVDKSRWQQGNVFSCSVMHEALHNHYTQKSLSLSPGGGSGGSEVQLLESGGGLVQPGGSLRLSCAASGFTFSNYAMSWFRQPPETGLKWVSSIDASGGDTYYADSVKGRFTISRDNSKNTLYLQMNSLRAEDTAVYYCAKEGSHGTDDSHYDVDVWGQGTTVTVSS

SEQ ID NO: 279 - protein, 578 aa, Artificial Sequence
  PR005839 Chain
QVQLVESGGGVVQPGRSLRLSCAASGFTFRSFGMHWVRQAPGKGLEWVAVISYDASNEYYADSVKGRFIISRDNSKDTLYLQMNSLRAGDTAVYYCAKGGGLRWYFAYWGQGTLVTVSSASTKGPSVFPLAPSSKSTSGGTAALGCLVKDYFPEPVTVSWNSGALTSGVHTFPAVLQSSGLYSLSSVVTVPSSSLGTQTYICNVNHKPSNTKVDKKVEPKSCDKTHTCPPCPAPELAGAPSVFLFPPKPKDTLMISRTPEVTCVVVDVSHEDPEVKFNWYVDGVEVHNAKTKPREEQYNSTYRVVSVLTVLHQDWLNGKEYKCKVSNKALPAPIEKTISKAKGQPREPQVYTLPPSREEMTKNQVSLTCLVKGFYPSDIAVEWESNGQPENNYKTTPPVLDSDGSFFLYSKLTVDKSRWQQGNVFSCSVMHEALHNHYTQKSLSLSPGGGSGGSEVQLLESGGGLVQPGGSLRLSCAASGFTFSNYAMSWFRQPPETGLKWVSSIDASGGDTYYADSVKGRFTISRDNSKNTLYLQMNSLRAEDTAVYYCAKEGSHGTDDSHYDVDVWGQGTTVTVSS

SEQ ID NO: 280 - protein, 578 aa, Artificial Sequence
  PR005866 Chain
QVQLVESGGGVVQPGRSLRLSCAASGFTFRSFGMHWVRQAPGKGLEWVAVISYDASNEYYADSVKGRFIISRDNSKDTLYLQMNSLRAGDTAVYYCAKGGGLRWYFAYWGQGTLVTVSSASTKGPSVFPLAPSSKSTSGGTAALGCLVKDYFPEPVTVSWNSGALTSGVHTFPAVLQSSGLYSLSSVVTVPSSSLGTQTYICNVNHKPSNTKVDKKVEPKSCDKTHTCPPCPAPELLGGPSVFLFPPKPKDTLMISRTPEVTCVVVDVSHEDPEVKFNWYVDGVEVHNAKTKPREEQYASTYRVVSVLTVLHQDWLNGKEYKCKVSNKALPAPIEKTISKAKGQPREPQVYTLPPSREEMTKNQVSLTCLVKGFYPSDIAVEWESNGQPENNYKTTPPVLDSDGSFFLYSKLTVDKSRWQQGNVFSCSVMHEALHNHYTQKSLSLSPGGGSGGSEVQLLESGGGLVQPGGSLRLSCAASGFTFSNYAMSWFRQPPETGLKWVSSIDASGGDTYYADSVKGRFTISRDNSKNTLYLQMNSLRAEDTAVYYCAKEGSHGTDDSHYDVDVWGQGTTVTVSS

SEQ ID NO: 281 - protein, 578 aa, Artificial Sequence
  PR007165 Chain
QVQLVESGGGVVQPGRSLRLSCAASGFTFRSFGMHWVRQAPGKGLEWVAVISYDASNEYYADSVKGRFIISRDNSKDTLYLQMNSLRAGDTAVYYCAKGGGLRWYFAYWGQGTLVTVSSASTKGPSVFPLAPSSKSTSGGTAALGCLVKDYFPEPVTVSWNSGALTSGVHTFPAVLQSSGLYSLSSVVTVPSSSLGTQTYICNVNHKPSNTKVDKKVEPKSCEVQLVESGGGVVQPGGSLRLSCAASGFTFSNYAMTWVRQAPEKGLEWVSSISGSGVSTYYADSVKGRFTISRDNSKNTLYLQMTRLTAEDTAVYFCAKEGSSETDDHYYNVDVWGQGTTVTVSSEPKSSDKTHTCPPCPAPEAAGGPSVFLFPPKPKDTLMISRTPEVTCVVVDVSHEDPEVKFNWYVDGVEVHNAKTKPREEQYNSTYRVVSVLTVLHQDWLNGKEYKCKVSNKALPAPIEKTISKAKGQPREPQVYTLPPSREEMTKNQVSLTCLVKGFYPSDIAVEWESNGQPENNYKTTPPVLDSDGSFFLYSKLTVDKSRWQQGNVFSCSVMHEALHNHYTQKSLSLSPGK

SEQ ID NO: 282 - protein, 12 aa, Artificial Sequence
  human IgG2 hinge
ERKCCVECPPCP

SEQ ID NO: 283 - protein, 19 aa, Artificial Sequence
  PR007381 HFWR2 Chothia
AMSWVRQAPGKGLEWVSSI

SEQ ID NO: 284 - protein, 124 aa, Artificial Sequence
  PR007381 VH
EVQLLESGGGLVQPGGSLRLSCAASGFTFSNYAMSWVRQAPGKGLEWVSSIDASGGDTYYADSVKGRFTISRDNSKNTLYLQMNSLRAEDTAVYYCAKEGSHGTDDSHYDVDVWGQGTTVTVSS

SEQ ID NO: 285 - protein, 356 aa, Artificial Sequence
  PR007381 HC
EVQLLESGGGLVQPGGSLRLSCAASGFTFSNYAMSWVRQAPGKGLEWVSSIDASGGDTYYADSVKGRFTISRDNSKNTLYLQMNSLRAEDTAVYYCAKEGSHGTDDSHYDVDVWGQGTTVTVSSEPKSCDKTHTCPPCPAPELLGGPSVFLFPPKPKDTLMISRTPEVTCVVVDVSHEDPEVKFNWYVDGVEVHNAKTKPREEQYNSTYRVVSVLTVLHQDWLNGKEYKCKVSNKALPAPIEKTISKAKGQPREPQVYTLPPSREEMTKNQVSLTCLVKGFYPSDIAVEWESNGQPENNYKTTPPVLDSDGSFFLYSKLTVDKSRWQQGNVFSCSVMHEALHNHYTQKSLSLSPGK

SEQ ID NO: 286 - protein, 578 aa, Artificial Sequence
  PR007379 Chain
QVQLVESGGGVVQPGRSLRLSCAASGFTFRSFGMHWVRQAPGKGLEWVAVISYDASNEYYADSVKGRFTISRDNSKDTLYLQMNSLRAEDTAVYYCAKGGGLRWYFAYWGQGTLVTVSSASTKGPSVFPLAPSSKSTSGGTAALGCLVKDYFPEPVTVSWNSGALTSGVHTFPAVLQSSGLYSLSSVVTVPSSSLGTQTYICNVNHKPSNTKVDKKVEPKSCDKTHTCPPCPAPEAAGGPSVFLFPPKPKDTLMISRTPEVTCVVVDVSHEDPEVKFNWYVDGVEVHNAKTKPREEQYNSTYRVVSVLTVLHQDWLNGKEYKCKVSNKALPAPIEKTISKAKGQPREPQVYTLPPSREEMTKNQVSLTCLVKGFYPSDIAVEWESNGQPENNYKTTPPVLDSDGSFFLYSKLTVDKSRWQQGNVFSCSVMHEALHNHYTQKSLSLSPGGGSGGSEVQLLESGGGLVQPGGSLRLSCAASGFTFSNYAMSWFRQPPETGLKWVSSIDASGGDTYYADSVKGRFTISRDNSKNTLYLQMNSLRAEDTAVYYCAKEGSHGTDDSHYDVDVWGQGTTVTVSS

SEQ ID NO: 287 - protein, 578 aa, Artificial Sequence
  PR007380 Chain
QVQLVESGGGVVQPGRSLRLSCAASGFTFRSFGMHWVRQAPGKGLEWVAVISYDASNEYYADSVKGRFTISRDNSKDTLYLQMNSLRAEDTAVYYCAKGGGLRWYFAYWGQGTLVTVSSASTKGPSVFPLAPSSKSTSGGTAALGCLVKDYFPEPVTVSWNSGALTSGVHTFPAVLQSSGLYSLSSVVTVPSSSLGTQTYICNVNHKPSNTKVDKKVEPKSCDKTHTCPPCPAPEAAGGPSVFLFPPKPKDTLMISRTPEVTCVVVDVSHEDPEVKFNWYVDGVEVHNAKTKPREEQYNSTYRVVSVLTVLHQDWLNGKEYKCKVSNKALPAPIEKTISKAKGQPREPQVYTLPPSREEMTKNQVSLTCLVKGFYPSDIAVEWESNGQPENNYKTTPPVLDSDGSFFLYSKLTVDKSRWQQGNVFSCSVMHEALHNHYTQKSLSLSPGGGSGGSEVQLLESGGGLVQPGGSLRLSCAASGFTFSNYAMSWVRQAPGKGLEWVSSIDASGGDTYYADSVKGRFTISRDNSKNTLYLQMNSLRAEDTAVYYCAKEGSHGTDDSHYDVDVWGQGTTVTVSS

SEQ ID NO: 288 - protein, 6 aa, Artificial Sequence
  (G2S)2
GGSGGS

SEQ ID NO: 289 - protein, 10 aa, Artificial Sequence
  (G4S)2
GGGGSGGGGS

SEQ ID NO: 290 - protein, 449 aa, Artificial Sequence
  ÖØÁ´ÐòÁÐ
QVQLVESGGGVVQPGRSLRLSCAASGFTFRSFGMHWVRQAPGKGLEWVAVISYDASNEYYADSVKGRFIISRDNSKDTLYLQMNSLRAGDTAVYYCAKGGALRWYFAYWGQGTLVTVSSASTKGPSVFPLAPSSKSTSGGTAALGCLVKDYFPEPVTVSWNSGALTSGVHTFPAVLQSSGLYSLSSVVTVPSSSLGTQTYICNVNHKPSNTKVDKKVEPKSCDKTHTCPPCPAPELLGGPDVFLFPPKPKDTLMISRTPEVTCVVVDVSHEDPEVKFNWYVDGVEVHNAKTKPREEQYNSTYRVVSVLTVLHQDWLNGKEYKCKVSNKALPAPEEKTISKAKGQPREPQVYTLPPSREEMTKNQVSLTCLVKGFYPSDIAVEWESNGQPENNYKTTPPVLDSDGSFFLYSKLTVDKSRWQQGNVFSCSVMHEALHNHYTQKSLSLSPGK

SEQ ID NO: 291 - protein, 215 aa, Artificial Sequence
  ÇáÁ´ÐòÁÐ
EIVMTQSPATLSVSPGERATLSCRASQSISSNLGWYQQKPGQAPRLLIYGASTRATGIPARFSGSGSGTEFTLTISSLQSEDFAVYYCQQYRSWPPLTFGGGTKVEIKRTVAAPSVFIFPPSDEQLKSGTASVVCLLNNFYPREAKVQWKVDNALQSGNSQESVTEQDSKDSTYSLSSTLTLSKADYEKHKVYACEVTHQGLSSPVTKSFNRGEC